European Patent Specification EP 3 091 078 B1, published November 26, 2025. Title: COMPOSITIONS, METHODS, AND PLANT GENES FOR THE IMPROVED PRODUCTION OF FERMENTABLE SUGARS FOR BIOFUEL PRODUCTION. Applicant: The Governing Council of the University of Toronto. Application New Divisional application based on EP13770094.4. The sequence listing filed with the application follows.

SEQUENCE LISTING (37 sequences)

SEQ ID NO: 1 - DNA, 1651 bp, Zea mays
tcgtcctcgctcggagacacggcaagcgagtcctcctcactcacgcaaacacacgccgtgccgcgagcgcacgagacaaccgagcggagctgccgcctgcccgccagtgccagccatggacgccgcggtgcgcgtccccccggcgctcgggaacaagacggtgaccgaggtgacgccgccgccgccaccaccggcgggggaggagcggctgtcggacgccgacacgacggcgtcgtcgacggcggcgcccaactcgagcctcagctcggccagcagcgccgccagcctgccgcgctgctccagcctgtcccgcctctccttcgactgctctccgtccgcggccctgtcctcttcctcggcggcggcggcggccgcggccgcgtcatcgccggcgccagcgccggcgcggccgcaccgggcaggggacgcggcgtgggcggcgatccgcgcggcgtcggcgtcggccgcggcgccgctggggccgcgggacttcaggctgctgcgccgcgtgggcggcggcgacgtcggcaccgtgtacctgtgccgcctcagggcgccacccgcgcccgcgcccgtctgctgcctgtacgcgatgaaggtggtggaccggcgcgtggcggccgcgaagaagaagctggagcacgcggcggcggagcggcggatcctgcgggcgctggaccatccgttcctgcccacgctcttcgccgacttcgacgccgcgccgcacttctcctgcgtcgtcacggagttctgccccggcggggacctccactcgctccgccaccgcatgcccaaccgccgcttcccgctcccgtcagctcggttctacgcggcggaggtgttgctggcgctggagtacctgcacatgatgggcatcgtgtaccgcgacctcaagccggagaacgtgctgatccgcgcggacggccacatcatgctcacggacttcgacctgtcgctgcagtgcacgtcgacgccgtcgctcgagccgtgcgccgcccccgaggcggcggcggcgtcctgcttcccggaccacctgttccgccgccggcgcgcgcgactccgccgtgccgcctcggcgcggcggccgccaacgaccctggtggcggagccggtggaggcgcggtcgtgctcgttcgtgggcacgcacgagtacgtggcgcccgaggtggcccgcggcgggccccacggcgcggccgtcgactggtgggcgctcggcgtgttcctgtacgagctcctgcacgggcgcaccccgttcgcgggcgccgacaacgaggccacgctccgcaacatcgcgcgccgcccgctgtccttccccgctgccggcgccggtgatgccgacgcgcgcgacctcatcgcccgcctcctcgccaaggacccgcgccaccggttggggtcccggcgcggcgccgccgacgtgaaggcgcacccgttcttccgcgggctcaacttcgcgctgctccggtcctcccgcccgcccgtcgtccccgccgcgtcgcgctccccgctgcaccgctcgcagtcctgcagcgcggcgcgcacgagagcgtcgaagccgaagccgccgccggacacccggttcgacctgttctgacacgaccgttgccggcgtcacgcacgtgcgtgttgacctagttgcatcactcgccattgt

SEQ ID NO: 2 - protein, 491 aa, Zea mays
MDAAVRVPPALGNKTVTEVTPPPPPPAGEERLSDADTTASSTAAPNSSLSSASSAASLPRCSSLSRLSFDCSPSAALSSSSAAAAAAAASSPAPAPARPHRAGDAAWAAIRAASASAAAPLGPRDFRLLRRVGGGDVGTVYLCRLRAPPAPAPVCCLYAMKVVDRRVAAAKKKLEHAAAERRILRALDHPFLPTLFADFDAAPHFSCVVTEFCPGGDLHSLRHRMPNRRFPLPSARFYAAEVLLALEYLHMMGIVYRDLKPENVLIRADGHIMLTDFDLSLQCTSTPSLEPCAAPEAAAASCFPDHLFRRRRARLRRAASARRPPTTLVAEPVEARSCSFVGTHEYVAPEVARGGPHGAAVDWWALGVFLYELLHGRTPFAGADNEATLRNIARRPLSFPAAGAGDADARDLIARLLAKDPRHRLGSRRGAADVKAHPFFRGLNFALLRSSRPPVVPAASRSPLHRSQSCSAARTRASKPKPPPDTRFDLF

SEQ ID NO: 3 - DNA, 958 bp, Zea mays
caaagccaacagaactgcacagtgtagtagttgcacataggcgtccgcgcgtcgtcctagctatggatccatatcactaccaaaccatgtatgacccacgcggcttccccatcatccacccgcagccttacctccagcacccggtggccggcgccctcggtgacagcagggtgcgcggcggcggcagtggcgcgcggcggcgtcctggcgccaagctctccacggacccgcagagcgttgcggcgcgcgagcggcggcaccgcatcagcgaccgcttccgcgtgctccgcagcctcgtccccggcggcagcaagatggacactgtgtccatgctcgagcaggccatccactacgtcaagttcctcaagacgcagatcagcctgcatcaggccgcgctgatgcagcacgaggaaggatgccatgctgagctcgccgcctattccgcggtggcggtggttggtgacaacgaggtgacactcgcgtcccatggtcgtaccggcgcatgcgacgagatgatgcagctccaggtggcggcggaggaagctttgagttatggtgttgatgcccatcagccgtacgggctcgatcccaggcagctgagtggtgggcacgagctgccaccgctgcctgcttcttgcatcttcctcgaggagcctgcagacgcatgctactctgtgtgtgacctcgacgacggggacaccggtctgcccggctcttactagagtagtagtagaagtttcttaaggtagcatcccgtgtgtgttggtgtctgctagacgctagtacgtctaattagcaaagtttagctagtactcgatcaattgtctgtctagttcgctcagagttaaagtatatgatgatgcatctgcatatatgggctctgtaattctgttatccgctgatcgcagatgatacaccgtatgtaatcacatgtatgtatgttgcctaaaaaaaaaaa

SEQ ID NO: 4 - protein, 219 aa, Zea mays
MDPYHYQTMYDPRGFPIIHPQPYLQHPVAGALGDSRVRGGGSGARRRPGAKLSTDPQSVAARERRHRISDRFRVLRSLVPGGSKMDTVSMLEQAIHYVKFLKTQISLHQAALMQHEEGCHAELAAYSAVAVVGDNEVTLASHGRTGACDEMMQLQVAAEEALSYGVDAHQPYGLDPRQLSGGHELPPLPASCIFLEEPADACYSVCDLDDGDTGLPGSY

SEQ ID NO: 5 - protein, 1646 aa, Arabidopsis thaliana
MDLHPPGGSKKTSVVVVTLDTGEVYVIASLLSKADTQVIYIDPTTGILRYNGKPGLDNFKSEREALDYITNGSRGGVRSSVYARAILGYAVLGSFGMLLVATRLNPSIPDLPGGGCVYTVAESQWVKIPLYNPQPQGKGETKNIQELTELDIDGKHYFCDTRDITRPFPSRMPLQSPDDEFVWNRWLSVPFKNIGLPEHCVILLQGFAEYRPFGSSGQLEGIVALMARRSRLHPGTRYLARGINSCSGTGNEVECEQLVWIPKRNGQSIAFNSYIWRHGTIPIWWGAELKMTAAEAEIYVADRDPYKGSTEYYQRLSKRYDTRNLDAPVGENQKKKAFVPIVCVNLLRSGEGKSECILVQHFEESMNFIKSSGKLPYTRVHLINYDWHASVKLKGEQQTIEGLWMYLKSPTMAIGISEGDYLPSRQRLKDCRGEVICIDDIEGAFCLRSHQNGVIRFNCADSLDRTNAASFFGGLQVFVEQCRRLGISLDTDLGYGHNSVNNQGGYNAPLPPGWEKRADAVTGKSYYIDHNTKTTTWSHPCPDKPWKRLDMRFEEFKRSTILSPVSELADLFLQQGDIHATLYTGSKAMHSQILNIFSEESGAFKQFSAAQKNMKITLQRRYKNAMVDSSRQKQLEMFLGMRLFKHLPSIPVQPLHVLSRPSGFFLKPVPNMSESSNDGSSLLSIKRKDITWLCPQAADIVELFIYLSEPCHVCQLLLTISHGADDLTCPSTVDVRTGRHIEDLKLVVELVQLDYRLPVIMFSGQGASIPRCANGTNLLVPLPGPISSEDMAVTGAGARLHEKDTSSLSLLYDFEELEGQLDFLTRVVAVTFYPAGAVRIPMTLGQIEVLGISLPWKGMFTCERTGGRLAELARKPDEDGSPFSSCSDLNPFAATTSLQAETVSTPVQQKDPFPSNLLDLLTGEDSSSDPFPQPVVECIASGGNDMLDFLDEAVVEYRGSDTVPDGSVPQNKRPKDSGAHLYLNCLKSLAGPNMAKKLEFVEAMKLEIERLRLNISAAERDRALLSIGIDPATINPNSSYDELYIGRLCKIANALAVMGQASLEDKIIASIGLEKLENNVIDFWNITRIGEGCDGGMCQVRAEVNKSPVGSSTKSSRGESGSVFLCFQCMKKACKFCCAGKGALLLSKSYSRDTANGGGSLADVSATSIGSDHYICKKCCSSIVLEALIVDYVRVMVSLRRSGRVDNAGREALNEVFGSNITNHLAVRGQPSPNREDFNFLRQILGKEESLSEFPFASFLHKVETATDSAPFFSLLTPLNLASSNAYWKAPPSADSVEAAIVLNTLSDVSSVILLVSPCGYSDADAPTVQIWASSDINKEARTLMGKWDVQSFIRSSPELSGSEKSGRAPRHIKFAFKNPVRCRIIWITLRLPRLGSSSSVSLDKNINLLSLDENPFAPIPRRASFGATIENDPCIHAKHILVTGNTVRDKTLQSVESMSVRNWLDRAPRLNRFLIPLETERPMENDLVLELYLQPASPLAAGFRLDAFSAIKPRVTHSPSSDVVDIWDPTSVIMEDRHVSPAILYIQVSVLQEQYKMVTIAEYRLPEARDGTKLYFDFPKQIQAQRVSFKLLGDVAAFTDEPAEAVDLSSRASPFAAGLSLANRIKLYYYADPYEVGKWTSLSSV

SEQ ID NO: 6 - DNA, 6394 bp, Arabidopsis thaliana
atggatctgcatccaccaggttagtttctttttgaagattcaagtgtttttttttttcactctagctgttttcatcatttggttggctaattttcttatcttcttggtgtaggtggttcaaaaaagacatctgtagttgttgtcaccttagacactggtgaagtctatgtcattgcaagtttgttatctaaggctgatactcaagttatctatatcgatcctacgactggtatcctgcggtacaatgggaagcctggccttgataattttaagtcagagcgtgaagccttagattatattacgaatggatcaagaggaggtgttagaagctctgtttatgccagggcaatactcggttatgctgtcttggggagctttgggatgcttttagttgcgaccaggctaaatccaagtattccagatttgcctggtggtggatgtgtatatacagtggctgagagtcaatgggtcaaaataccactctacaatccacagcctcaagggaaaggtgaaaccaagaatattcaggagttgactgagcttgacatcgacgggaagcactatttctgtgatactagagacatcactcggcccttcccaagccgtatgccacttcaaagccctgatgatgaatttgtttggaatagatggttgtccgtgccttttaagaatattgggctacctgaacactgtgtcattcttctgcaggttcgtcctccattaatgaattgatgaaggttgatctacctatccgatttcggttttgtgtgaagattcaaaagcatataaattgatatgacatcatcttcttatttgatgttaattataggggtttgcagaatatcgaccttttgggagctcaggccagctagaagggattgttgctctaatggcccgtcgtagcagactgcatccagggactcgttacctagctaggggcattaattcatgttctggcacaggtgacatgcccccctaaaatgctcctctctcttaatttctttgttgttctcttaaaaagtgtggctctggattgactagggcctaatttagaagtatatgtgtagtgcaggtaacgaagttgagtgtgagcagcttgtatggatacctaaaagaaatggtcaaagcattgctttcaactcgtacatttggcgacatggcaccataccaatatggtggggtgcagaattaaagatgactgcggcagaagcagaaatttatgtggcagatagggatccttataaaggcagtacagagtattaccaaaggttaagcaagcgatatgatactaggaatctagatgcacctgttggagaaaaccagaagaaaaaggcttttgttcctattgtgtgcgttaatttactaagaagtggagaagggaaatcagaatgtatcttagtacaacattttgaagaatcgatgaactttatcaaatccagtggaaagcttccttatactcgtgttcacctgataaattatgattggcatgccagcgtgaaactaaaaggggaacagcaaactattgaaggattgtggatgtatctaaaatctcccactatggcaataggaatttctgaaggtgactatttgccttcacgtcaaagactgaaagattgcagaggtgaggtaatctgtattgatgacattgaaggtgccttctgtttgagatcacatcaaaatggggtgatacgttttaactgcgctgattccttggatcgaacaaatgcggctagtttctttggtggtcttcaagtgtttgtagagcaatgtagaaggctgggaatatcacttgatactgatcttggatatggtcataattctgttaataatcaggggggatataacgctccccttccaccgggatgggaaaaaagagctgatgccgtaactggaaaatcatattatatagatcacaatacaaagacaacaacatggagtcatccatgtcctgataaaccatggaagagacttgacatgaggtttgaggaatttaagagatcaactatcttatctcctgtgtcagaacttgccgatctttttctgcaacaaggtgatatccatgcaaccctctatactggctcgaaagctatgcacagccaaattctcaacatcttcagtgaagaatcaggagcatttaaacagttttctgcagcacagaaaaacatgaagattacactacagagaagatataaaaatgctatggttgatagttcacggcaaaaacagctcgagatgtttctgggaatgaggcttttcaagcatcttccatcaattcctgtccagcctttacatgtaagcacattgacacgattccagtaaaaaattcccagctctcagctctccttttttccatgtatattaactgctctaaagtatgaatcacgtttttttgcgtgtatgtagattttgtttcatattggaccgatacactttgtttattgtgtgtagatatataattcctaagagcataacagattcgttgatttgtagactctactatttgttgctttctatattctctgtctacttctcactgcaaaaatattcatgtcaggtactttctcgaccatctggtttctttctgaaacctgtacctaacatgtccgaaagttccaatgatgggtccagtctgctgagtatcaagaggaaggacataacttgggtacctcaacttagatataagattacctcttagttctcattacttgaatacttgagctaaaaaaattccatgctttttgttacttttgcagctatgtccacaagctgcagatattgttgaattatttatctatctcagtgagccttgccatgtatgtcaacttctactgaccatatcacacggtgcggatgatttgacatgtccatccactgtggacgtgagaactggacgccacatagaggaccttaaattagttgttgaggttgactctcttttaggtcttgtcccttctgttttattgtttgtaggagatctgtagacttacatgcaagttagttcaactggattaccgattacctgtaattatgttttctggacagggtgcttcaataccacgctgtgcaaatggtacaaatcttctggtacccttaccagggccaattagttctgaggatatggctgttactggagctggtgcacgtcttcatgaaaaagatacgtcaagtctttcactgctatatgattttgaagaactagaaggacagttggatttcttaacccgtgtagttgctgttacattttatccagctggtgctgttagaattcctatgactcttggtcaggtacttactagtttccaaactatgaattgatgaatatctattagcttcatcatgctctgaactcgttaaagtttatgattagctatcatcaaaagaagaaaaaacaaacactttttctgcattgtgtctatgccgcagatagaagtccttggaatttctcttccatggaaaggaatgtttacttgtgaacgtactggaggaagattagctgaacttgcaaggaaaccagatgaagatggaagtcctttttcatcttgttctgacttgaatccgtttgctgcaacaacatctttacaggctgaaactgtttccacaccagtacaacagaaggatccctttcccagtaatctgcttgaccttttgacaggagaggactcttcttctgaccccttcccacaaccagtggtggaatgtattgcaagtggaggcaatgacatgcttgatttcttagacgaagcagttgttgaatatcgcggctctgacactgttcctgacgggtctgtcccacaaaataaaaggcccaaggacagtggtgctcatctgtacttaaattgcctaaagtcccttgcgggtccaaacatggtgagatgcaattacgtctttccagttgccacaaactgtagttctgattgtatgaatctttcattggtttaactattcttctcatatgttatctttcttcgtaaaattccattttctatggtaaatttaatttctgcatgtctggcataatacaggcaaagaagcttgagtttgtagaagctatgaagcttgaaattgaacgtctacgtctcaatatttctgcagcagaaagagatagggcactgttatcgattggaattgatccagctaccattaatccaaactcttcatacgacgagttatatattggaagattatgcaaaatagcaaatgcacttgcagttatgggccaggcttctcttgaagataaaattatagcttctattggtctagagaagctggaaaataatgtgatagatttctggaacataaccagaattggtgagggttgtgatggcggaatgtgtcaagtccgagccgaggtcaataaaagtccagttggatcttctaccaagagttcaagaggagagtcgggctcagtgttcttgtgcttccaatgtatgaaaaaagcttgcaagttttgttgtgctggaaaaggagctcttctgctttcaaaatcctactccagggacactgcgaatggaggtggaagtcttgcagatgtctctgctacttcgataggttcagatcattacatttgtaaaaaatgctgcagctcgatagtgcttgaagccctgattgtagattatgtaagggtcatggtcagcttgcgaagaagtggccgtgttgataatgctggtcgggaagctttgaatgaggtatttggatctaacattacaaatcaccttgctgttagaggtcaaccttctcctaatcgagaagacttcaatttccttcgtcaaattttgggtaaagaggagtcgctttctgagttcccatttgcaagcttcttacataaggtaatatgcttcttatgtgttttaaaattactatgatcacttcattgtctttggaaagagctgttatgtaatacctaatcctcctttctctcttttggatgtttgcataatgcaatttaggtcgaaactgcgactgattcagcaccatttttctcattgctcacccctctgaatcttgcttcaagtaatgcctactggaaagctcctccgtctgcagactctgttgaagccgccattgttctcaacaccctttcagatgtcagcagtgtgattctactcgttagtccatgtggttactctgatgctgatgctcctaccgtaagtttgacttttctatcttcagttgaattcttgttaacccatgccattacttacgtgataatgctgccactcatttcaacattttatgtatcttcattgcaggtccaaatttgggcgagcagcgacataaacaaggaagcacggactttgatgggaaagtgggatgtacagtcctttattagatcttcgcctgagctttctggttcagaaaagtctggtagagcacctaggcatataaaatttgctttcaagaatcctgtccgttgccgcattatatggataacactgcgtcttcctaggcttggatctagtagctcagttagtttggacaaaaacatcaatctcttatctttggatgagaacccatttgctccaattcctcgacgtgcctcttttggagcaaccattgagaatgatccatgtattcatgcaaaacacatcttggtcactggaaacaccgtgagggataaaacgctacaaagtgttgagagcatgagcgtaagaaactggctggacagagccccacgtttgaatagattcctggttagtgccttagagaactgctcgttccttttcacctttttctgtggtatttcgtttattgtcactaatatttgtttttttcaccttccagataccattagagactgagagaccaatggagaatgatctagtcttggaactttatctgcaacctgcttcacctttagctgctggattccgtttagatgcttttagtgcgataaagcctcgtgtaacccactcgccttcttcagatgtagttgacatttgggacccgacgagtgtcataatggaagatagacacgtctctccggccatcttgtatatacaagtatctgttctacaggtatctatctctcctcctcccggtttattatatatcctcagaaaccaaaatgttgtaataactttttcatgttgatctgaaaaatgttaatctacaggagcaatacaaaatggtgacaatcgcggaatacagattgcctgaggcgagagatggaacaaagttgtattttgacttccctaaacagatacaagcacagagagtatcgtttaaactgctaggagatgtagcagcttttacagatgagcccgcagaggctgttgatttgagcagccgggcttctccttttgctgcaggactgtctttagcaaacaggatcaagctatattactatgcggatccttacgaagtaggcaaatggactagcctttcaagtgtctga

SEQ ID NO: 7 - protein, 438 aa, Arabidopsis thaliana
MLRESDGEMSLGTTNSPISSGTESCSSFSRLSFDAPPSTIPEEESFLSLKPHRSSDFAYAEIRRRKKQGLTFRDFRLMRRIGAGDIGTVYLCRLAGDEEESRSSYFAMKVVDKEALALKKKMHRAEMEKTILKMLDHPFLPTLYAEFEASHFSCIVMEYCSGGDLHSLRHRQPHRRFSLSSARFYAAEVLVALEYLHMLGIIYRDLKPENILVRSDGHIMLSNFDLSLCSDSIAAVESSSSSPENQQLRSPRRFTRLARLFQRVLRSKKVQTLEPTRLFVAEPVTARSGSFVGTHEYVAPEVASGGSHGNAVDWWAFGVFLYEMIYGKTPFVAPTNDVILRNIVKRQLSFPTDSPATMFELHARNLISGLLNKDPTKRLGSRRGAAEVKVHPFFKGLNFALIRTLTPPEIPSSVVKKPMKSATFSGRSSNKPAAFDYF

SEQ ID NO: 8 - DNA, 1624 bp, Arabidopsis thaliana
atgttacgagaatcagacggtgagatgagtttaggaacaacaaactcaccgataagcagcggaacagagagttgcagcagtttcagccggttatcattcgacgcgccgccgtcaactatccccgaagaagaaagcttcctttctctcaaacctcaccgatcctcagatttcgcttacgcagagatccgaagacgaaaaaaacaaggcctaaccttccgagattttcgcctcatgcgtcgtatcggcgccggcgacatcggaacagtttacttatgccgtctagccggagacgaagaagagagccggagctcgtattttgcgatgaaagttgtggataaagaagctcttgcgttgaagaagaagatgcatagagcagagatggagaaaacgattttgaaaatgcttgaccatccatttttgccgactctttacgctgagtttgaagcctcacatttctcttgcatcgttatggaatattgctccggtggtgatttacactctctccgtcatagacaacctcaccggcgattctccctctcttccgccaggtaaaaaatatcaaattttattgaataatttaatattatggacaaagtcagattttttttcaaaaaaaaaaaattgtgaaaaaagattcatcatcatcaatgtatatatatattttatagttacatgcattgactctgttcacatttgttatcttgttctgcaagaacagacctgttcttatcatgtcggtcttttccagttctttgaattgttatcaaagagtctttttcagcccatcacaatttataaacgtcaataattatgattttattagctaatgagtatttattttgtttttggttacagattttatgccgccgaagttctagtggcgttagaatatctacacatgttgggtatcatctacagagatctgaagcctgaaaatatcttagttagatccgacggtcacattatgctctctaactttgacctctctctatgctccgactcaatcgcagccgttgaatcttcctcgtcttcgccggagaatcaacaactccgttcaccgcgacgattcactcgtctcgctagacttttccaacgagtcttgcggtctaaaaaggttcagactttagaaccaacccgtctctttgttgctgaaccggttactgcccggtccggttcgttcgttggtacgcatgaatacgtggcaccagaagttgcttcaggtggatcacatggtaatgccgttgactggtgggcctttggagtgtttctctacgagatgatatatggcaagactccgttcgttgcgccgactaatgacgtcattctccgtaacattgtgaaaagacagttgagtttcccgactgattcgccggcgactatgtttgagcttcatgcgcggaatttgatttccgggttgcttaacaaagatccgactaaaagacttgggtcacggcgaggtgcggcggaggttaaagtgcatccttttttcaaaggtctaaactttgcgctcattcgtacgcttactccgccggagattccttcttccgtcgtcaagaagccgatgaaatcggcgacgtttagtggtagaagtagtaacaaaccagcggcgttcgattacttttga

SEQ ID NO: 9 - protein, 322 aa, Arabidopsis thaliana
MMNLGSLSLSTSKSSKPMVSISFWIPYFTHWGESLLVCGSAPGLGSGNVKKGLLLKPSQQDDQLIWSGSVSVPPGFSSDYCYYVVDDSKSVLRSEFGMKRKLVVPETLTGGESVHLRDLWQSGDQALPFRSAFKDVIFHHSFDVKVEKPLGVFMNKSDQDDSVVVQFKICCPDIGEGTSVYVLGTPEKLGNWKVENGLRLNYVDDSIWEADCLIPKADFPIKYRYCKVQKEDSIGFESGGNRELSLHSIGSKQEYIVMSDGLFRAMPWRGAGVAVPMFSVRSEDDVGVGEFLDLKLLVDWAVDSGLHLVQLLPVNDTSVHKM

SEQ ID NO: 10 - DNA, 5412 bp, Arabidopsis thaliana
atgatgaatctaggatctctttcgttgagtacgagcaagtcgagtaagccaatggttagcatcagcttttggataccgtatttcactcactggggagagagcctgctggtctgtggctcggctcctggacttggttccgggaatgtgaaaaaaggtttgctgctaaagccatcccagcaagatgatcagctcatctggagtggctctgtctcggttccacctgggtttagctctgactattgttactatgtggtggatgactcgaagagtgtgttaaggtcggagtttgggatgaaacgaaaacttgtggtgcctgagacattgaccggtggagagtctgttcatcttcgtgatctctggcaggtttgagttctttgtccttttcgagtgtattatacaaattttgtaatctgattttgtagtgttgtgattgatgttctgttcctttaattttagagtggggatcaagctcttccatttagaagtgcatttaaagatgtcatcttccaccacagtttcgatgtgaaagtagaaaaacctctaggggtctttatgaataagtcagatcaagatggtattcatttttttatctaatcctatcacaccattgtctctgagattctctagtttgtgattgatctctttgctaactgttgtggccttatgactttaccatgtaaacagattcagttgttgtccaattcaaaatctgttgtccagacattggagagggaacatctgtaagcctttctctatgatctttggttttctttcttttcatgtttgagcctgatgtggtgttgtggccatcattcttacccttgattatgacatgtacaggtgtatgttctaggcaccccagaaaagttggggaattggaaagttgaaaatggacttagactcaactatgtcgatgattccatatgggaagcagattgcttgatccctaaagcagactttcctatcaaatatcctttctttttactttcttccagactaattagttgaacatagttgacacttcacttctcatatgctttctgcatgttgggttcttaacgattctttcacatatagatactgtaaagttcagaaggaagatagcatagggtttgaatctggtggtaatcgggagctgtctcttcactccatcggtagtaaacaggaatacattgtcatgtcagatggcttgtttcgagtaagtaacagagacaagctatgaactagctctaatgtgacagaatcaatgttgtcttactattatttaattttacttgtaggcaatgccatggaggggtgctggtgtagcagttcccatgttctctgtaaggtcagaagatgatgttggtgtgggagagtttctcgatctgaagttgcttgttgattgggctgtagattccgggttgcatctagtacaacttttaccagtaaatgacacatccgttcataagatgtgatgggactcgtatccctacaggtatgatgattacatttatgttagttttgcaggagttcaataaaggacttctgtcacttacttaacggatggaaacaaatatccagaatttttgttattattctttcttgactactgaattcataaatagttcattttttgcttcaatttggttttcgagaccttgggttccatatactttggttgatgattagtgactgagcctgaggctctgctgaatattagtctctactctctacttagtaaaatttctatatcaactcattgaactgtgtgattcattcttattgttcctttcctcatttggattgcttctcttgcagctcgttatctgtgtttgcattgcatccattatatcttagagtgcaggctctctctgaacgtctgccagaagatatcaaggtaagtttctacacttattgtatcctggaagagactcctaagcaatatattggctgacctttttcgttctctttcaggaagaaattcagaaggcgaagaatcaactggacaagaatgtaatgagtcccttgttagacgtttcatagattttcttacttttacgtccttgaaaaagatagcatcagataaacgggatatagtatttttaaatggtttgtgtctgtatcagcatgatgtgtttaaacgcctgcaagcaattggttcatatgttagttcgtcacaatcagagtttgagtgttgtaacctaatcctttaaagattgttacgtgtaggatgttgattatgaggctaccatggaaactaagctttcaattgccaagaaaatctttgacatagagaaagaccagactttgaactcaagcaccttccagaaattcttctctgaaaacgaggtatgcttcaaaatctgatattgtttccttgatatctcttgagaattgtctgcatagaacttatgcctccaaaggccacgtcagcgttccattggcttacggatttttgttatctttgaaagggctggttgaaaccatatgcagctttctgcttccttcgtgacttttttgagacttcagatcatagtcagtgggggaccttttctgactatacagacgacaaggtataatttgcttttatgttgttcaagtttaagttgtgatcgaattagttcaagctttccagatgtatttcatatagtttcagtaatttctcacatctccaaataacatttgccacagcttgaaaaattgatatccaaggacaacttgcactataacactatatgcttccactactacattcagtaccatttacatgtacaagtaagtatgttctgatttatctagttatattccattcttgtaagtgaagtcggttactggatgtttcatctaaagtgtgttctggttccattttcaaaagttgtcagcagcagcagaatatgcaaggaagaaaggagttgtgctgaaaggagacctacctattggcgttgacagaaacagtgttgatacgtgggtttacaggaatctgtttcgcatgaatacgtcaactggagcacctccagactattttgacaaaaatggtcagaactggggatttcctacttataactgggaggaaatgtcaaaagacaactatgcctggtggcgtgctcgcctaacacaggttggaattattgtccttaccagccacatcctttgtagatctgaaggctgaccacattgcatacttgctttgcagatggggaaatatttcacagcatacaggattgatcatatattgggattcttcagaatctgggagcttccagctcatgctatgactggtttagtggggaagttccgtccatctattcctttaagtcaggtacacaagctacatgcttacagttaaaaaaaacttggctttgagagttacttgatgataaaactgctgctgatgcaggaagagttggaaaaggagggaatatgggattttgaccgcttaagcaagccctatatccagaagaagtttcttgaggttagttttccatcacatttattatgatctgcctctgtcacagcttagttagtttgtgagttttcaatctcattacctatttgttgataatatgtcattgttctgttccttcaggagaaatttggagatttttggccttttattgcatcaaactttcttaatgaaactcagaaggacatgtatgaggttagtaaaaatcctcatttagagatcgttttcctttggagaaccaagtcttacctttttctgtccaaaactctgtggtgttttttgctaagtggatgtattaaatctttcttaattggtttcctttaattgtactctagttcaaggaggactgcaacacagagaagaagattgtagcaaagctgaagtcattggctgagaagtctttgttgctagaaaatgaggacaaagttcgacgtgatgtctttgacattttacgggtaaactttcatgcatcacaagggctttccagatttcttctccttgttatataaagtgactctgtccacttcacgtctctctcaagtccactgtcccaattgtttatttctgttgaacttgtgtccctagaatgttgttctgatcaaagatccagaggatgcaagaaaattctatcctcgctttaatattgaggatacttcaagcttccaggatttggatgatcacaggtacattcaaaaccttttcccagtcacttcccaaatagagtagtctgctcttgttcctttgattttatatcgcccatgaacatttacacagatcctctcttgctattgtatcgtgctgtatttttctacttttcatcaatatgggaaaatctgattaaggttttctcatacagcaaaaatgttctgaagaggctatactatgactactatttccaacgccaagaggatctatggagaaaaaatgctttgaaaaccttgcctgctctgttgaattcatctaatatgctggcatgtggggaggatctgggtctcattccatcttgtgtacatcctgtatgtgctctgttttctttctcttggttcatccaacttctttataaaacttgtgtagaagcatatgctaaaattaatagttactcaggttatgcaagaactgggattggttggccttcgcatccagcgcatgccaagtgagtccgatgtgaagtttgggattccgtctaattatgactatatgacggttagatatttttcctcagacttctgtctttcttacttatagcttcctaccgttcattttctgagaattttgtaatgggtgagtgattcactgcataattcaaactatcgtcttaatattttaggtgtgtgctccttcatgccacgactgctctaccctgcgagcttggtgggaagaggacgaagagagaagacagcagtacttcaaggaagtgattggtgtagatggaatccctccaagtcagtgtattccagagataactcatttcattctgaggcaacatgttgaagctccatcaatgtgggctattttcccgcttcaggtaatcatcaccactgtccgacttctcagatttattagaactttttatgaggctcaataacagtatgtgttgtttgtttttttcctctggaacaatttaggatatgatggctctgaaagaagagtacactactcgtcctgcaacagaggagacaatcaatgatccaacaaaccccaaacactactggagataccgtaagtatttactactaactaacacacaaccctaagaactataccagttttaacttagactgttttttgtgcatataggcgtacacgtgactttggactcgcttctaaaggacactgacctgaagtcaaccatcaagaacctcgtttccagcagtggaagatctgttcctgctaatgtttctggtgaagacatcaacaaaagccgaggagaagttatagccaatggctcgactaagccaaacccataa

SEQ ID NO: 11 - protein, 955 aa, Arabidopsis thaliana
MMNLGSLSLSTSKSSKPMVSISFWIPYFTHWGESLLVCGSAPGLGSGNVKKGLLLKPSQQDDQLIWSGSVSVPPGFSSDYCYYVVDDSKSVLRSEFGMKRKLVVPETLTGGESVHLRDLWQSGDQALPFRSAFKDVIFHHSFDVKVEKPLGVFMNKSDQDDSVVVQFKICCPDIGEGTSVYVLGTPEKLGNWKVENGLRLNYVDDSIWEADCLIPKADFPIKYRYCKVQKEDSIGFESGGNRELSLHSIGSKQEYIVMSDGLFRAMPWRGAGVAVPMFSVRSEDDVGVGEFLDLKLLVDWAVDSGLHLVQLLPVNDTSVHKMWWDSYPYSSLSVFALHPLYLRVQALSERLPEDIKEEIQKAKNQLDKNDVDYEATMETKLSIAKKIFDIEKDQTLNSSTFQKFFSENEGWLKPYAAFCFLRDFFETSDHSQWGTFSDYTDDKLEKLISKDNLHYNTICFHYYIQYHLHVQLSAAAEYARKKGVVLKGDLPIGVDRNSVDTWVYRNLFRMNTSTGAPPDYFDKNGQNWGFPTYNWEEMSKDNYAWWRARLTQMGKYFTAYKIDHILGFFRIWELPAHAMTGLVGKFRPSIPLSQEELEKEGIWDFDRLSKPYIQKKFLEEKFGDFWPFIASNFLNETQKDMYEFKEDCNTEKKIVAKLKSLAEKSLLLENEDKVRRDVFDILRNVVLIKDPEDARKFYPRFNIEDTSSFQDLDDHSKNVLKRLYYDYYFQRQEDLWRKNALKTLPALLNSSNMLACGEDLGLIPSCVHPVMQELGLVGLRIQRMPSESDVKFGIPSNYDYMTVCAPSCHDCSTLRAWWEEDEERRQQYFKEVIGVDGIPPSQCIPEITHFILRQHVEAPSMWAIFPLQDMMALKEEYTTRPATEETINDPTNPKHYWRYRVHVTLDSLLKDTDLKSTIKNLVSSSGRSVPANVSGEDINKSRGEVIANGSTKPNP

SEQ ID NO: 12 - DNA, 5412 bp, Arabidopsis thaliana
atgatgaatctaggatctctttcgttgagtacgagcaagtcgagtaagccaatggttagcatcagcttttggataccgtatttcactcactggggagagagcctgctggtctgtggctcggctcctggacttggttccgggaatgtgaaaaaaggtttgctgctaaagccatcccagcaagatgatcagctcatctggagtggctctgtctcggttccacctgggtttagctctgactattgttactatgtggtggatgactcgaagagtgtgttaaggtcggagtttgggatgaaacgaaaacttgtggtgcctgagacattgaccggtggagagtctgttcatcttcgtgatctctggcaggtttgagttctttgtccttttcgagtgtattatacaaattttgtaatctgattttgtagtgttgtgattgatgttctgttcctttaattttagagtggggatcaagctcttccatttagaagtgcatttaaagatgtcatcttccaccacagtttcgatgtgaaagtagaaaaacctctaggggtctttatgaataagtcagatcaagatggtattcatttttttatctaatcctatcacaccattgtctctgagattctctagtttgtgattgatctctttgctaactgttgtggccttatgactttaccatgtaaacagattcagttgttgtccaattcaaaatctgttgtccagacattggagagggaacatctgtaagcctttctctatgatctttggttttctttcttttcatgtttgagcctgatgtggtgttgtggccatcattcttacccttgattatgacatgtacaggtgtatgttctaggcaccccagaaaagttggggaattggaaagttgaaaatggacttagactcaactatgtcgatgattccatatgggaagcagattgcttgatccctaaagcagactttcctatcaaatatcctttctttttactttcttccagactaattagttgaacatagttgacacttcacttctcatatgctttctgcatgttgggttcttaacgattctttcacatatagatactgtaaagttcagaaggaagatagcatagggtttgaatctggtggtaatcgggagctgtctcttcactccatcggtagtaaacaggaatacattgtcatgtcagatggcttgtttcgagtaagtaacagagacaagctatgaactagctctaatgtgacagaatcaatgttgtcttactattatttaattttacttgtaggcaatgccatggaggggtgctggtgtagcagttcccatgttctctgtaaggtcagaagatgatgttggtgtgggagagtttctcgatctgaagttgcttgttgattgggctgtagattccgggttgcatctagtacaacttttaccagtaaatgacacatccgttcataagatgtggtgggactcgtatccctacaggtatgatgattacatttatgttagttttgcaggagttcaataaaggacttctgtcacttacttaacggatggaaacaaatatccagaatttttgttattattctttcttgactactgaattcataaatagttcattttttgcttcaatttggttttcgagaccttgggttccatatactttggttgatgattagtgactgagcctgaggctctgctgaatattagtctctactctctacttagtaaaatttctatatcaactcattgaactgtgtgattcattcttattgttcctttcctcatttggattgcttctcttgcagctcgttatctgtgtttgcattgcatccattatatcttagagtgcaggctctctctgaacgtctgccagaagatatcaaggtaagtttctacacttattgtatcctggaagagactcctaagcaatatattggctgacctttttcgttctctttcaggaagaaattcagaaggcgaagaatcaactggacaagaatgtaatgagtcccttgttagacgtttcatagattttcttacttttacgtccttgaaaaagatagcatcagataaacgggatatagtatttttaaatggtttgtgtctgtatcagcatgatgtgtttaaacgcctgcaagcaattggttcatatgttagttcgtcacaatcagagtttgagtgttgtaacctaatcctttaaagattgttacgtgtaggatgttgattatgaggctaccatggaaactaagctttcaattgccaagaaaatctttgacatagagaaagaccagactttgaactcaagcaccttccagaaattcttctctgaaaacgaggtatgcttcaaaatctgatattgtttccttgatatctcttgagaattgtctgcatagaacttatgcctccaaaggccacgtcagcgttccattggcttacggatttttgttatctttgaaagggctggttgaaaccatatgcagctttctgcttccttcgtgacttttttgagacttcagatcatagtcagtgggggaccttttctgactatacagacgacaaggtataatttgcttttatgttgttcaagtttaagttgtgatcgaattagttcaagctttccagatgtatttcatatagtttcagtaatttctcacatctccaaataacatttgccacagcttgaaaaattgatatccaaggacaacttgcactataacactatatgcttccactactacattcagtaccatttacatgtacaagtaagtatgttctgatttatctagttatattccattcttgtaagtgaagtcggttactggatgtttcatctaaagtgtgttctggttccattttcaaaagttgtcagcagcagcagaatatgcaaggaagaaaggagttgtgctgaaaggagacctacctattggcgttgacagaaacagtgttgatacgtgggtttacaggaatctgtttcgcatgaatacgtcaactggagcacctccagactattttgacaaaaatggtcagaactggggatttcctacttataactgggaggaaatgtcaaaagacaactatgcctggtggcgtgctcgcctaacacaggttggaattattgtccttaccagccacatcctttgtagatctgaaggctgaccacattgcatacttgctttgcagatggggaaatatttcacagcatacaagattgatcatatattgggattcttcagaatctgggagcttccagctcatgctatgactggtttagtggggaagttccgtccatctattcctttaagtcaggtacacaagctacatgcttacagttaaaaaaaacttggctttgagagttacttgatgataaaactgctgctgatgcaggaagagttggaaaaggagggaatatgggattttgaccgcttaagcaagccctatatccagaagaagtttcttgaggttagttttccatcacatttattatgatctgcctctgtcacagcttagttagtttgtgagttttcaatctcattacctatttgttgataatatgtcattgttctgttccttcaggagaaatttggagatttttggccttttattgcatcaaactttcttaatgaaactcagaaggacatgtatgaggttagtaaaaatcctcatttagagatcgttttcctttggagaaccaagtcttacctttttctgtccaaaactctgtggtgttttttgctaagtggatgtattaaatctttcttaattggtttcctttaattgtactctagttcaaggaggactgcaacacagagaagaagattgtagcaaagctgaagtcattggctgagaagtctttgttgctagaaaatgaggacaaagttcgacgtgatgtctttgacattttacgggtaaactttcatgcatcacaagggctttccagatttcttctccttgttatataaagtgactctgtccacttcacgtctctctcaagtccactgtcccaattgtttatttctgttgaacttgtgtccctagaatgttgttctgatcaaagatccagaggatgcaagaaaattctatcctcgctttaatattgaggatacttcaagcttccaggatttggatgatcacaggtacattcaaaaccttttcccagtcacttcccaaatagagtagtctgctcttgttcctttgattttatatcgcccatgaacatttacacagatcctctcttgctattgtatcgtgctgtatttttctacttttcatcaatatgggaaaatctgattaaggttttctcatacagcaaaaatgttctgaagaggctatactatgactactatttccaacgccaagaggatctatggagaaaaaatgctttgaaaaccttgcctgctctgttgaattcatctaatatgctggcatgtggggaggatctgggtctcattccatcttgtgtacatcctgtatgtgctctgttttctttctcttggttcatccaacttctttataaaacttgtgtagaagcatatgctaaaattaatagttactcaggttatgcaagaactgggattggttggccttcgcatccagcgcatgccaagtgagtccgatgtgaagtttgggattccgtctaattatgactatatgacggttagatatttttcctcagacttctgtctttcttacttatagcttcctaccgttcattttctgagaattttgtaatgggtgagtgattcactgcataattcaaactatcgtcttaatattttaggtgtgtgctccttcatgccacgactgctctaccctgcgagcttggtgggaagaggacgaagagagaagacagcagtacttcaaggaagtgattggtgtagatggaatccctccaagtcagtgtattccagagataactcatttcattctgaggcaacatgttgaagctccatcaatgtgggctattttcccgcttcaggtaatcatcaccactgtccgacttctcagatttattagaactttttatgaggctcaataacagtatgtgttgtttgtttttttcctctggaacaatttaggatatgatggctctgaaagaagagtacactactcgtcctgcaacagaggagacaatcaatgatccaacaaaccccaaacactactggagataccgtaagtatttactactaactaacacacaaccctaagaactataccagttttaacttagactgttttttgtgcatataggcgtacacgtgactttggactcgcttctaaaggacactgacctgaagtcaaccatcaagaacctcgtttccagcagtggaagatctgttcctgctaatgtttctggtgaagacatcaacaaaagccgaggagaagttatagccaatggctcgactaagccaaacccataa

SEQ ID NO: 13 - DNA, 3576 bp, Arabidopsis thaliana
atgaattgtcttcagaatcttcccaggtatcttcttgctttccgaaattagcaaatgttgttgatttgtgtggttctttgattcgatatgaatttgtgtgttgttgatgtctttgatcgtcatttatttcagatgttcagtctcacctctgctgggattcgggtgcattcaaagagatcattcttcttcttcttcttctttgaagatgctaatatcgcctccgatcaaagccaatgatccaaaatctcgacttgttttacatgtatacacctcttttaagatatattgttatatcagtttttttcttctaacttttattgacacttttgtaaatgctttgagtgtaggcagtatcagagtcaaaatccagctcagagatgagtggtgttgcaaaggatgaagagaaatctgatgaatatagccaagacatgactcaagctatgggtgctggtaaattgttttcatcatacctatacatgtccttagattggaaactctaatgatgtccaccattttttgtctcatattggaaatattgatttagctcattggattgtattctactcttgtttttcatctttcatcttgattagttttgttcatctgtctaccaaggaatcttatatcttttgcttgtttattgacaaacttatcttcttgttctccttaattatgtatttcagtcactgattcattctcatgtgtctttcatttcagttctaacttacaggcacgagttaggaatgaactacaactttattcgtccagatctaattgttggatcctgcttacaggttcacttttatatccttctctcaaatgatgattttgttttggatatgtggtactttcctcgtgttcttactgtatgctctcctttattgctagacccctgaagatgttgacaagcttcgtaaaattggagttaaaaccatattttgcttgcaacaagatccagacctggagtatccttccaaagccctctttttctgttcatgattatgattttgttttcactttccttcgcattgagtgaggaagaatgatctgcagtgcagaatgccttgaccaatccttccagatattttggagtagacataagcagcatccaagcctatgctaagaaatatagtgatattcagcatattcgctgtgaaattaggtaaggcaacgatctagctgtgactttttaatatattggtattcaaagctgatgcgtaatgaatcgaaggagagatcatgagttgatttttagtttcctttccaatatttttcttattgcttgactttataagaagcatatgaggtagttttttttccagaattatctgaataggcgagggaacaaaggtatatacactgttggagggtagtctcagatatcttttaggcacgcaatctttaaattcttattgttttgtcagtgaagtgttatactttctttttctttgggctctttacttttatcacgtttcctaagctaatgggaaatcagcacacttttgtgtaagcaataactggtttatgacgaattgtgagtgatagtttttttttaccgggtgtgaaatcactgctatcaactaacttttttgttcgtccacctttgtctgtttacaaactagagtaactgtagaagttagtcatcatcccattctcactaaatttctttactgctaaagacttggaaccatcatcatcccttttggcatatatgagactgttcacgagcacatgcatagaaaaattcaccatggacgtacccactcacaacgtaggggattgacatattatatatcattgatgtaacagagactttgatgcatttgatttgagaatgcgtcttccagccgtggttggtactctttacaaagctgttaagcgaaatggaggagttacatatgtgcactgcactgctggaatgggaagggctcctgctgttgcggtatgttacagaaacctgttactaagctcttctctttttcccccttttctttccagtattgaaaaaatgtaagactgttgcaaacagtagttgtcttaattttgtgcttatttggttgactcatgaaggtatgaacaagttttcacattttgctgactgatactgagaagggatattaatttcattttcagttgacatacatgttctgggtgcaaggctataagcttatggaagctcataaattacttatgataagatactaatttacttgtggtttatgttctctatatgtgtttctttatacttatattaagtaaccaacatgttaatcatgttttactagtgttactgcctgttatattatgtgaggatgtttggggatttccttcttctcctatgaaccgacaattatgataactagaatcatagaccattgggtcaggggtttgtagtaaatatacactgaagatatagcactttaaaagacaaaaatcttgggttagttcatccaaaatagtctagcattagacatttttagtttgatatctctagatggctggtgaaacataaaggcacgcgtaaatttggtttatataacatttctgaaattttcttgcagagcaaaaggtcgtgctttccgaagctggatgctatcagaaatgcaacaattgatattgtgagtcagcgttcaactttcacaatgcttcctatgtttgaaaaacctcagttccattgattagcatgagtgcgcaacagttacctggttccttgactcctgattattgtttccgggtgtatatggataaaagcttacaggactcaagaggaagactgttactctgacactgaaagataaggggttctccagagtagaaatttctggccttgacattggatggggacaggtaaatatattttatcttaaaccaatttatttattatgacaccttgctcttaaatctatggtgtgccatataagctttaaagccaggatgcacttttgtcactgctattaaaagaatggcctctttgataagaagtggaagagatgagtgttggatttctgaaaattattgtcttatgattgtgcaaaactatttggacgtatatatataaaaggtaatgtatttctttagctcttttcgtttttaccatttttctctttatgtagaggatacctctaacactggacaagggaacaggattctggatcctaaagagagaactgcctgtgagttttcttcttaactgttaagcatagtgtctgatcattttccaacaaccactacaatttctgaaatgcaggaaggacagtttgaatataaatacatcatagatggtgaatggacacacaatgaggccgaaccgtttataggacctaacaaagacggccataccaacaattacgctaaagtaaaaatgtctctgtctcttaacatatagctgaacaagttttgatgaatgagttaatgctgtaatgttgttgtgtactaatgaattaggtagtggacgatccaacaagtgtggatggtacaactcgggagagactatcgagcgaagaccctgagctgttggaggaagaacgctcgaaactaatccagttcttggagacttgttctgaggcagaagtttga

SEQ ID NO: 14 - DNA, 5380 bp, Arabidopsis thaliana
atggaggccagtgccggcttggttgctggatcctaccggagaaacgagctcgttcggatccgacatgaatctgatggcggggtctgttcatcttccctttttcccatttttttgttattgtttttcgttcttacaatttttgatgtgtagatctcatctagatttctctgtttctaaatctcgtctcttttggatccataattggatcattgaaactcagatttcgcttcctttgactgtgtagttagttagtgtcagttgatcaagtaagtgtctgaaaatggaaacttttctgctccaattcttcaaattgttgtgatctatatcaattaatgccgcatctgttttcttaaaatctcttatggaaagtgtcggtggatttcagttcgttaacttttttaagctaaaatctttgactcttaaagtttagctttacttattgagatttagctcaactagatctcgttagttcccgccatgggatacagactgtgactcgccttaattcagatctgcattgattgttttgatttagatccttgctcatctctttctgtagtttctaatactcaatgactaacaatgatgcaatgttggtcaaagtgcagaccaaacctttgaagaatatgaatggccagatatgtcagatctgtggtgatgatgttggactcgctgaaactggagatgtctttgtcgcgtgtaatgaatgtgccttccctgtgtgtcggccttgctatgagtacgagaggaaagatggaactcagtgttgccctcaatgcaagactagattcagacgacacaggggtcagttgtctttttctttttgttggcaattgctatatatggattttctctttttgtttctttgctgttgtgttgaacaattttttggaattttccagggagtcctcgtgttgaaggagatgaagatgaggatgatgttgatgatatcgagaatgagttcaattacgcccagggagctaacaaggcgagacaccaacgccatggcgaagagttttcttcttcctctagacatgaatctcaaccaattcctcttctcacccatggccatacggtagggacctacattttccctttagactctagagtgatttgtattactcaataaatccctagagtggtcatttattacttactattcacgttaatgttatatgtgaacaaatcttaacagaatttttttctgatagtacatggtcatccaaattaagaaataataatagatgttgttagttgtgtctgttttcaatagattcatgacctttttctatacacaggtttctggagagattcgcacgcctgatacacaatctgtgcgaactacatcaggtcctttgggtccttctgacaggaatgctatttcatctccatatattgatccacggcaacctggtattcatatgtttttcccttgtgcacgtggtctttgttaaatgtgattcctattcatttttacaacatatatattttgtgtaccgtaactgatagctcccgctaaaaattgcagtccctgtaagaatcgtggacccgtcaaaagacttgaactcttatgggcttggtaatgttgactggaaagaaagagttgaaggctggaagctgaagcaggagaaaaatatgttacagatgactggtaaataccatgaagggaaaggaggagaaattgaagggactggttccaatggcgaagaactccaaatgtaagtggaaatactagaccaatatctttattgtccaactcaaacagctcttggccgtgatgctaataaccactcttggtttcttattatgtattgatagacataattaagtatctgctttgttacatttgtttccttccactcaattatggttctcgtacttacagggctgatgatacacgtcttcctatgagtcgtgtggtgcctatcccatcttctcgcctaaccccttatcgggttgtgattattctccggcttatcatcttgtgtttcttcttgcaatatcgtacaactcaccctgtgaaaaatgcatatcctttgtggttgacctcggttatctgtgagatctggtttgcattttcttggcttcttgatcagtttcccaaatggtaccccattaacagggagacttatcttgaccgtctcgctataaggttggtctttaagtttatacatcccctactctcatctctcttttatgtattaacttgatatcttctatcacagttttcgatagttgactttttccccctgtaaatttaatttaaatttagacaatggtgcatctgaattttgattatgatatatcttaagaagattatgattgtaaatcttgaaatttagtagaaaaccatctgcaatctactgaccatgtgaagtttccgactagactatgatagaagcatgccaagtggagtgtttattaagatagagcttagctattatactgattttatatgtgttttgattttttggtttcttattgtagatatgatcgagacggtgaaccatcacagctcgttcctgttgatgtgtttgttagtacagtggacccattgaaagagcctccccttgttacagcaaacacagttctctcgattctttctgtggactacccggtagataaagtagcctgttatgtttcagatgatggttcagctatgcttacctttgaatccctttctgaaaccgctgagtttgcaaagaaatgggtaccattttgcaagaaattcaacattgaacctagggcccctgaattctattttgcccagaagatagattacttgaaggacaagatccaaccgtcttttgttaaagagcgacgagctatgaaggtcatttgaaaagtccacctgcttctcatccatacggcaaagagattgactgactttttctttggtttgtattgacagagagagtatgaagagtttaaagtgaggataaatgctcttgttgccaaagcacagaaaatccctgaagaaggctggacaatgcaggatggtactccctggcctggtaacaacactagagatcatcctggaatgatacaggtacagtgtggcaatcccttgattgtgacagagaggataacgtaaaggaaacatgtttacatcgttttgtttcaatttcaggtgttcttaggccatagtgggggtctggataccgatggaaatgagctgcctagactcatctatgtttctcgtgaaaagcggcctggatttcaacaccacaaaaaggctggagctatgaatgcattggtttgttaactttcagaatcctattgtgtcctctattttattctcttgttcactgcctaagaaacgttcttcttgtgtagccgttgcttcacattcttttttttctaggctatgtgttctctcctaatttagtatctctttactttgacagatccgtgtatctgctgttcttaccaatggagcatatcttttgaacgtggattgtgatcattactttaataacagtaaggctattaaagaagctatgtgtttcatgatggacccggctattggaaagaagtgctgctatgtccagttccctcaacgttttgacggtattgatttgcacgatcgatatgccaacaggaatatagtctttttcgatgtgagtatcacttccccattgtcttttgtttctcttttgttcatattttggttggatttactcgtttctgctatggcctgacttggatatttgttctcttgggcagattaacatgaaggggttggatggtatccagggtccagtatatgtgggtactggttgttgttttaataggcaggctctatatgggtatgatcctgttttgacggaagaagatttagaaccaaatattattgtcaagagctgttgcgggtcaaggaagaaaggtaaaagtagcaagaagtataactacgaaaagaggagaggcatcaacagaagtgactccaatgctccacttttcaatatggaggacatcgatgagggttttgaaggtttgattgagctgattgtgtaataacatcacttctttatgtaatgatttatgtgatggtgaaatcttacaatccttgtttatgcaggttatgatgatgagaggtctattctaatgtcccagaggagtgtagagaagcgttttggtcagtcgccggtatttattgcggcaaccttcatggaacaaggcggcattccaccaacaaccaatcccgctactcttctgaaggaggctattcatgttataagctgtggttacgaagacaagactgaatggggcaaagaggtcagttttcaaatgcagctacagaatcttcttatgttctctttcttacctgtttgatgacatcttatttggcacttttgttagattggttggatctatggttccgtgacggaagatattcttactgggttcaagatgcatgcccggggttggatatcgatctactgcaatcctccacgccctgcgttcaagggatctgcaccaatcaatctttctgatcgtttgaaccaagttcttcgatgggctttgggatctatcgagattcttcttagcagacattgtcctatctggtatggttaccatggaaggttgagacttttggagaggatcgcttatatcaacaccatcgtctatcctattacatccatccctcttattgcgtattgtattcttcccgctttttgtctcatcaccgacagattcatcatacccgaggtttgtaaaactgaccacactgctatttactatttgaatcccattttgtgaatgcatttttttgtcatcatcattgttgcagataagcaactacgcgagtatttggttcattctactcttcatctcaattgctgtgactggaatcctggagctgagatggagcggtgtgagcattgaggattggtggaggaacgagcagttctgggtcattggtggcacatccgcccatctttttgctgtcttccaaggtctacttaaggttcttgctggtatcgacaccaacttcaccgttacatctaaagccacagacgaagatggggattttgcagaactctacatcttcaaatggacagctcttctcattccaccaaccaccgtcctacttgtgaacctcataggcattgtggctggtgtctcttatgctgtaaacagtggctaccagtcgtggggtccgcttttcaggaagctcttcttcgccttatgggttattgcccatctctaccctttcttgaaaggtctgttgggaagacaaaaccgaacaccaaccatcgtcattgtctggtctgttcttctcgcctccatcttctcgttgctttgggtcaggatcaatccctttgtggacgccaatcccaatgccaacaacttcaatggcaaaggaggtgtcttttag

SEQ ID NO: 15 - protein, 1081 aa, Arabidopsis thaliana
MEASAGLVAGSYRRNELVRIRHESDGGTKPLKNMNGQICQICGDDVGLAETGDVFVACNECAFPVCRPCYEYERKDGTQCCPQCKTRFRRHRGSPRVEGDEDEDDVDDIENEFNYAQGANKARHQRHGEEFSSSSRHESQPIPLLTHGHTVSGEIRTPDTQSVRTTSGPLGPSDRNAISSPYIDPRQPVPVRIVDPSKDLNSYGLGNVDWKERVEGWKLKQEKNMLQMTGKYHEGKGGEIEGTGSNGEELQMADDTRLPMSRVVPIPSSRLTPYRVVIILRLIILCFFLQYRTTHPVKNAYPLWLTSVICEIWFAFSWLLDQFPKWYPINRETYLDRLAIRYDRDGEPSQLVPVDVFVSTVDPLKEPPLVTANTVLSILSVDYPVDKVACYVSDDGSAMLTFESLSETAEFAKKWVPFCKKFNIEPRAPEFYFAQKIDYLKDKIQPSFVKERRAMKREYEEFKVRINALVAKAQKIPEEGWTMQDGTPWPGNNTRDHPGMIQVFLGHSGGLDTDGNELPRLIYVSREKRPGFQHHKKAGAMNALIRVSAVLTNGAYLLNVDCDHYFNNSKAIKEAMCFMMDPAIGKKCCYVQFPQRFDGIDLHDRYANRNIVFFDINMKGLDGIQGPVYVGTGCCFNRQALYGYDPVLTEEDLEPNIIVKSCCGSRKKGKSSKKYNYEKRRGINRSDSNAPLFNMEDIDEGFEGYDDERSILMSQRSVEKRFGQSPVFIAATFMEQGGIPPTTNPATLLKEAIHVISCGYEDKTEWGKEIGWIYGSVTEDILTGFKMHARGWISIYCNPPRPAFKGSAPINLSDRLNQVLRWALGSIEILLSRHCPIWYGYHGRLRLLERIAYINTIVYPITSIPLIAYCILPAFCLITDRFIIPEISNYASIWFILLFISIAVTGILELRWSGVSIEDWWRNEQFWVIGGTSAHLFAVFQGLLKVLAGIDTNFTVTSKATDEDGDFAELYIFKWTALLIPPTTVLLVNLIGIVAGVSYAVNSGYQSWGPLFRKLFFALWVIAHLYPFLKGLLGRQNRTPTIVIVWSVLLASIFSLLWVRINPFVDANPNANNFNGKGGVF

SEQ ID NO: 16 - DNA, 5380 bp, Arabidopsis thaliana
atggaggccagtgccggcttggttgctggatcctaccggagaaacgagctcgttcggatccgacatgaatctgatggcggggtctgttcatcttccctttttcccatttttttgttattgtttttcgttcttacaatttttgatgtgtagatctcatctagatttctctgtttctaaatctcgtctcttttggatccataattggatcattgaaactcagatttcgcttcctttgactgtgtagttagttagtgtcagttgatcaagtaagtgtctgaaaatggaaacttttctgctccaattcttcaaattgttgtgatctatatcaattaatgccgcatctgttttcttaaaatctcttatggaaagtgtcggtggatttcagttcgttaacttttttaagctaaaatctttgactcttaaagtttagctttacttattgagatttagctcaactagatctcgttagttcccgccatgggatacagactgtgactcgccttaattcagatctgcattgattgttttgatttagatccttgctcatctctttctgtagtttctaatactcaatgactaacaatgatgcaatgttggtcaaagtgcagaccaaacctttgaagaatatgaatggccagatatgtcagatctgtggtgatgatgttggactcgctgaaactggagatgtctttgtcgcgtgtaatgaatgtgccttccctgtgtgtcggccttgctatgagtacgagaggaaagatggaactcagtgttgccctcaatgcaagactagattcagacgacacaggggtcagttgtctttttctttttgttggcaattgctatatatggattttctctttttgtttctttgctgttgtgttgaacaattttttggaattttccagggagtcctcgtgttgaaggagatgaagatgaggatgatgttgatgatatcgagaatgagttcaattacgcccagggagctaacaaggcgagacaccaacgccatggcgaagagttttcttcttcctctagacatgaatctcaaccaattcctcttctcacccatggccatacggtagggacctacattttccctttagactctagagtgatttgtattactcaataaatccctagagtggtcatttattacttactattcacgttaatgttatatgtgaacaaatcttaacagaatttttttctgatagtacatggtcatccaaattaagaaataataatagatgttgttagttgtgtctgttttcaatagattcatgacctttttctatacacaggtttctggagagattcgcacgcctgatacacaatctgtgcgaactacatcaggtcctttgggtccttctgacaggaatgctatttcatctccatatattgatccacggcaacctggtattcatatgtttttcccttgtgcacgtggtctttgttaaatgtgattcctattcatttttacaacatatatattttgtgtaccgtaactgatagctcccgctaaaaattgcagtccctgtaagaatcgtggacccgtcaaaagacttgaactcttatgggcttggtaatgttgactggaaagaaagagttgaaggctggaagctgaagcaggagaaaaatatgttacagatgactggtaaataccatgaagggaaaggaggagaaattgaagggactggttccaatggcgaagaactccaaatgtaagtggaaatactagaccaatatctttattgtccaactcaaacagctcttggccgtgatgctaataaccactcttggtttcttattatgtattgatagacataattaagtatctgctttgttacatttgtttccttccactcaattatggttctcgtacttacagggctgatgatacacgtcttcctatgagtcgtgtggtgcctatcccatcttctcgcctaaccccttatcgggttgtgattattctccggcttatcatcttgtgtttcttcttgcaatatcgtacaactcaccctgtgaaaaatgcatatcctttgtggttgacctcggttatctgtgagatctggtttgcattttcttggcttcttgatcagtttcccaaatggtaccccattaacagggagacttatcttgaccgtctcgctataaggttggtctttaagtttatacatcccctactctcatctctcttttatgtattaacttgatatcttctatcacagttttcgatagttgactttttccccctgtaaatttaatttaaatttagacaatggtgcatctgaattttgattatgatatatcttaagaagattatgattgtaaatcttgaaatttagtagaaaaccatctgcaatctactgaccatgtgaagtttccgactagactatgatagaagcatgccaagtggagtgtttattaagatagagcttagctattatactgattttatatgtgttttgattttttggtttcttattgtagatatgatcgagacggtgaaccatcacagctcgttcctgttgatgtgtttgttagtacagtggacccattgaaagagcctccccttgttacagcaaacacagttctctcgattctttctgtggactacccggtagataaagtagcctgttatgtttcagatgatggttcagctatgcttacctttgaatccctttctgaaaccgctgagtttgcaaagaaatgggtaccattttgcaagaaattcaacattgaacctagggcccctgaattctattttgcccagaagatagattacttgaaggacaagatccaaccgtcttttgttaaagagcgacgagctatgaaggtcatttgaaaagtccacctgcttctcatccatacggcaaagagattgactgactttttctttggtttgtattgacagagagagtatgaagagtttaaagtgaggataaatgctcttgttgccaaagcacagaaaatccctgaagaaggctggacaatgcaggatggtactccctggcctggtaacaacactagagatcatcctggaatgatacaggtacagtgtggcaatcccttgattgtgacagagaggataacgtaaaggaaacatgtttacatcgttttgtttcaatttcaggtgttcttaggccatagtgggggtctggataccgatggaaatgagctgcctagactcatctatgtttctcgtgaaaagcggcctggatttcaacaccacaaaaaggctggagctatgaatgcattggtttgttaactttcagaatcctattgtgtcctctattttattctcttgttcactgcctaagaaacgttcttcttgtgtagccgttgcttcacattcttttttttctaggctatgtgttctctcctaatttagtatctctttactttgacagatccgtgtatctgctgttcttaccaatggagcatatcttttgaacgtggattgtgatcattactttaataacagtaaggctattaaagaagctatgtgtttcatgatggacccggctattggaaagaagtgctgctatgtccagttccctcaacgttttgacggtattgatttgcacgatcgatatgccaacaggaatatagtctttttcgatgtgagtatcacttccccattgtcttttgtttctcttttgttcatattttggttggatttactcgtttctgctatggcctgacttggatatttgttctcttgggcagattaacatgaaggggttggatggtatccagggtccagtatatgtgggtactggttgttgttttaataggcaggctctatatgggtatgatcctgttttgacggaagaagatttagaaccaaatattattgtcaagagctgttgcgggtcaaggaagaaaggtaaaagtagcaagaagtataactacgaaaagaggagaggcatcaacagaagtgactccaatgctccacttttcaatatggaggacatcgatgagggttttgaaggtttgattgagctgattgtgtaataacatcacttctttatgtaatgatttatgtgatggtgaaatcttacaatccttgtttatgcaggttatgatgatgagaggtctattctaatgtcccagaggagtgtagagaagcgttttggtcagtcgccggtatttattgcggcaaccttcatggaacaaggcggcattccaccaacaaccaatcccgctactcttctgaaggaggctattcatgttataagctgtggttacgaagacaagactgaatggggcaaagaggtcagttttcaaatgcagctacagaatcttcttatgttctctttcttacctgtttgatgacatcttatttggcacttttgttagattggttggatctatggttccgtgacggaagatattcttactgggttcaagatgcatgcccggggttggatatcgatctactgcaatcctccacgccctgcgttcaagggatctgcaccaatcaatctttctgatcgtttgaaccaagttcttcgatgggctttgggatctatcgagattcttcttagcagacattgtcctatctggtatggttaccatggaaggttgagacttttggagaggatcgcttatatcaacaccatcgtctatcctattacatccatccctcttattgcgtattgtattcttcccgctttttgtctcatcaccgacagattcatcatacccgaggtttgtaaaactgaccacactgctatttactatttgaatcccattttgtgaatgcatttttttgtcatcatcattgttgcagataagcaactacgcgagtatttggttcattctactcttcatctcaattgctgtgactggaatcctggagctgagatggagcggtgtgagcattgaggattggtggaggaacgagcagttctgggtcattggtggcacatccgcccatctttttgctgtcttccaaggtctacttaaggttcttgctggtatcgacaccaacttcaccgttacatctaaagccacagacgaagatggggattttgcagaactctacatcttcaaatggacagctcttctcattccaccaaccaccgtcctacttgtgaacctcataggcattgtggctggtgtctcttatgctgtaaacagtggctaccagtcgtggggtctgcttttcgggaagctcttcttcgccttatgggttattgcccatctctaccctttcttgaaaggtctgttgggaagacaaaaccgaacaccaaccatcgtcattgtctggtctgttcttctcgcctccatcttctcgttgctttgggtcaggatcaatccctttgtggacgccaatcccaatgccaacaacttcaatggcaaaggaggtgtcttttag

SEQ ID NO: 17 - protein, 1081 aa, Arabidopsis thaliana
MEASAGLVAGSYRRNELVRIRHESDGGTKPLKNMNGQICQICGDDVGLAETGDVFVACNECAFPVCRPCYEYERKDGTQCCPQCKTRFRRHRGSPRVEGDEDEDDVDDIENEFNYAQGANKARHQRHGEEFSSSSRHESQPIPLLTHGHTVSGEIRTPDTQSVRTTSGPLGPSDRNAISSPYIDPRQPVPVRIVDPSKDLNSYGLGNVDWKERVEGWKLKQEKNMLQMTGKYHEGKGGEIEGTGSNGEELQMADDTRLPMSRVVPIPSSRLTPYRVVIILRLIILCFFLQYRTTHPVKNAYPLWLTSVICEIWFAFSWLLDQFPKWYPINRETYLDRLAIRYDRDGEPSQLVPVDVFVSTVDPLKEPPLVTANTVLSILSVDYPVDKVACYVSDDGSAMLTFESLSETAEFAKKWVPFCKKFNIEPRAPEFYFAQKIDYLKDKIQPSFVKERRAMKREYEEFKVRINALVAKAQKIPEEGWTMQDGTPWPGNNTRDHPGMIQVFLGHSGGLDTDGNELPRLIYVSREKRPGFQHHKKAGAMNALIRVSAVLTNGAYLLNVDCDHYFNNSKAIKEAMCFMMDPAIGKKCCYVQFPQRFDGIDLHDRYANRNIVFFDINMKGLDGIQGPVYVGTGCCFNRQALYGYDPVLTEEDLEPNIIVKSCCGSRKKGKSSKKYNYEKRRGINRSDSNAPLFNMEDIDEGFEGYDDERSILMSQRSVEKRFGQSPVFIAATFMEQGGIPPTTNPATLLKEAIHVISCGYEDKTEWGKEIGWIYGSVTEDILTGFKMHARGWISIYCNPPRPAFKGSAPINLSDRLNQVLRWALGSIEILLSRHCPIWYGYHGRLRLLERIAYINTIVYPITSIPLIAYCILPAFCLITDRFIIPEISNYASIWFILLFISIAVTGILELRWSGVSIEDWWRNEQFWVIGGTSAHLFAVFQGLLKVLAGIDTNFTVTSKATDEDGDFAELYIFKWTALLIPPTTVLLVNLIGIVAGVSYAVNSGYQSWGLLFGKLFFALWVIAHLYPFLKGLLGRQNRTPTIVIVWSVLLASIFSLLWVRINPFVDANPNANNFNGKGGVF

SEQ ID NO: 18 - DNA, 5380 bp, Arabidopsis thaliana
atggaggccagtgccggcttggttgctggatcctaccggagaaacgagctcgttcggatccgacatgaatctgatggcggggtctgttcatcttccctttttcccatttttttgttattgtttttcgttcttacaatttttgatgtgtagatctcatctagatttctctgtttctaaatctcgtctcttttggatccataattggatcattgaaactcagatttcgcttcctttgactgtgtagttagttagtgtcagttgatcaagtaagtgtctgaaaatggaaacttttctgctccaattcttcaaattgttgtgatctatatcaattaatgccgcatctgttttcttaaaatctcttatggaaagtgtcggtggatttcagttcgttaacttttttaagctaaaatctttgactcttaaagtttagctttacttattgagatttagctcaactagatctcgttagttcccgccatgggatacagactgtgactcgccttaattcagatctgcattgattgttttgatttagatccttgctcatctctttctgtagtttctaatactcaatgactaacaatgatgcaatgttggtcaaagtgcagaccaaacctttgaagaatatgaatggccagatatgtcagatctgtggtgatgatgttggactcgctgaaactggagatgtctttgtcgcgtgtaatgaatgtgccttccctgtgtgtcggccttgctatgagtacgagaggaaagatggaactcagtgttgccctcaatgcaagactagattcagacgacacaggggtcagttgtctttttctttttgttggcaattgctatatatggattttctctttttgtttctttgctgttgtgttgaacaattttttggaattttccagggagtcctcgtgttgaaggagatgaagatgaggatgatgttgatgatatcgagaatgagttcaattacgcccagggagctaacaaggcgagacaccaacgccatggcgaagagttttcttcttcctctagacatgaatctcaaccaattcctcttctcacccatggccatacggtagggacctacattttccctttagactctagagtgatttgtattactcaataaatccctagagtggtcatttattacttactattcacgttaatgttatatgtgaacaaatcttaacagaatttttttctgatagtacatggtcatccaaattaagaaataataatagatgttgttagttgtgtctgttttcaatagattcatgacctttttctatacacaggtttctggagagattcgcacgcctgatacacaatctgtgcgaactacatcaggtcctttgggtccttctgacaggaatgctatttcatctccatatattgatccacggcaacctggtattcatatgtttttcccttgtgcacgtggtctttgttaaatgtgattcctattcatttttacaacatatatattttgtgtaccgtaactgatagctcccgctaaaaattgcagtccctgtaagaatcgtggacccgtcaaaagacttgaactcttatgggcttggtaatgttgactggaaagaaagagttgaaggctggaagctgaagcaggagaaaaatatgttacagatgactggtaaataccatgaagggaaaggaggagaaattgaagggactggttccaatggcgaagaactccaaatgtaagtggaaatactagaccaatatctttattgtccaactcaaacagctcttggccgtgatgctaataaccactcttggtttcttattatgtattgatagacataattaagtatctgctttgttacatttgtttccttccactcaattatggttctcgtacttacagggctgatgatacacgtcttcctatgagtcgtgtggtgcctatcccatcttctcgcctaaccccttatcgggttgtgattattctccggcttatcatcttgtgtttcttcttgcaatatcgtacaactcaccctgtgaaaaatgcatatcctttgtggttgacctcggttatctgtgagatctggtttgcattttcttggcttcttgatcagtttcccaaatggtaccccattaacagggagacttatcttgaccgtctcgctataaggttggtctttaagtttatacatcccctactctcatctctcttttatgtattaacttgatatcttctatcacagttttcgatagttgactttttccccctgtaaatttaatttaaatttagacaatggtgcatctgaattttgattatgatatatcttaagaagattatgattgtaaatcttgaaatttagtagaaaaccatctgcaatctactgaccatgtgaagtttccgactagactatgatagaagcatgccaagtggagtgtttattaagatagagcttagctattatactgattttatatgtgttttgattttttggtttcttattgtagatatgatcgagacggtgaaccatcacagctcgttcctgttgatgtgtttgttagtacagtggacccattgaaagagcctccccttgttacagcaaacacagttctctcgattctttctgtggactacccggtagataaagtagcctgttatgtttcagatgatggttcagctatgcttacctttgaatccctttctgaaaccgctgagtttgcaaagaaatgggtaccattttgcaagaaattcaacattgaacctagggcccctgaattctattttgcccagaagatagattacttgaaggacaagatccaaccgtcttttgttaaagagcgacgagctatgaaggtcatttgaaaagtccacctgcttctcatccatacggcaaagagattgactgactttttctttggtttgtattgacagagagagtatgaagagtttaaagtgaggataaatgctcttgttgccaaagcacagaaaatccctgaagaaggctggacaatgcaggatggtactccctggcctggtaacaacactagagatcatcctggaatgatacaggtacagtgtggcaatcccttgattgtgacagagaggataacgtaaaggaaacatgtttacatcgttttgtttcaatttcaggtgttcttaggccatagtgggggtctggataccgatggaaatgagctgcctagactcatctatgtttctcgtgaaaagcggcctggatttcaacaccacaaaaaggctggagctatgaatgcattggtttgttaactttcagaatcctattgtgtcctctattttattctcttgttcactgcctaagaaacgttcttcttgtgtagccgttgcttcacattcttttttttctaggctatgtgttctctcctaatttagtatctctttactttgacagatccgtgtatctgctgttcttaccaatggagcatatcttttgaacgtggattgtgatcattactttaataacagtaaggctattaaagaagctatgtgtttcatgatggacccggctattggaaagaagtgctgctatgtccagttccctcaacgttttgacggtattgatttgcacgatcgatatgccaacaggaatatagtctttttcgatgtgagtatcacttccccattgtcttttgtttctcttttgttcatattttggttggatttactcgtttctgctatggcctgacttggatatttgttctcttgggcagattaacatgaaggggttggatggtatccagggtccagtatatgtgggtactggttgttgttttaataggcaggctctatatgggtatgatcctgttttgacggaagaagatttagaaccaaatattattgtcaagagctgttgcgggtcaaggaagaaaggtaaaagtagcaagaagtataactacgaaaagaggagaggcatcaacagaagtgactccaatgctccacttttcaatatggaggacatcgatgagggttttgaaggtttgattgagctgattgtgtaataacatcacttctttatgtaatgatttatgtgatggtgaaatcttacaatccttgtttatgcaggttatgatgatgagaggtctattctaatgtcccagaggagtgtagagaagcgttttggtcagtcgccggtatttattgcggcaaccttcatggaacaaggcggcattccaccaacaaccaatcccgctactcttctgaaggaggctattcatgttataagctgtggttacgaagacaagactgaatggggcaaagaggtcagttttcaaatgcagctacagaatcttcttatgttctctttcttacctgtttgatgacatcttatttggcacttttgttagattggttggatctatggttccgtgacggaagatattcttactgggttcaagatgcatgcccggggttggatatcgatctactgcaatcctccacgccctgcgttcaagggatctgcaccaatcaatctttctgatcgtttgaaccaagttcttcgatgggctttgggatctatcgagattcttcttagcagacattgtcctatctggtatggttaccatggaaggttgagacttttggagaggatcgcttatatcaacaccatcgtctatcctattacatccatccctcttattgcgtattgtattcttcccgctttttgtctcatcaccgacagattcatcatacccgaggtttgtaaaactgaccacactgctatttactatttgaatcccattttgtgaatgcatttttttgtcatcatcattgttgcagataagcaactacgcgagtatttggttcattctactcttcatctcaattgctgtgactggaatcctggagctgagatggagcggtgtgagcattgaggattggtggaggaacgagcagttctgggtcattggtggcacatccgcccatctttttgctgtcttccaaggtctacttaaggttcttgctggtatcgacaccaacttcaccgttacatctaaagccacagacgaagatggggattttgcagaactctacatcttcaaatggacagctcttctcattccaccaaccaccgtcctacttgtgaacctcataggcattgtggctggtgtctcttatgctgtaaacagtggctaccagtcgtgggatccgcttttcgggaagctcttcttcgccttatgggttattgcccatctctaccctttcttgaaaggtctgttgggaagacaaaaccgaacaccaaccatcgtcattgtctggtctgttcttctcgcctccatcttctcgttgctttgggtcaggatcaatccctttgtggacgccaatcccaatgccaacaacttcaatggcaaaggaggtgtcttttag

SEQ ID NO: 19 - protein, 1081 aa, Arabidopsis thaliana
MEASAGLVAGSYRRNELVRIRHESDGGTKPLKNMNGQICQICGDDVGLAETGDVFVACNECAFPVCRPCYEYERKDGTQCCPQCKTRFRRHRGSPRVEGDEDEDDVDDIENEFNYAQGANKARHQRHGEEFSSSSRHESQPIPLLTHGHTVSGEIRTPDTQSVRTTSGPLGPSDRNAISSPYIDPRQPVPVRIVDPSKDLNSYGLGNVDWKERVEGWKLKQEKNMLQMTGKYHEGKGGEIEGTGSNGEELQMADDTRLPMSRVVPIPSSRLTPYRVVIILRLIILCFFLQYRTTHPVKNAYPLWLTSVICEIWFAFSWLLDQFPKWYPINRETYLDRLAIRYDRDGEPSQLVPVDVFVSTVDPLKEPPLVTANTVLSILSVDYPVDKVACYVSDDGSAMLTFESLSETAEFAKKWVPFCKKFNIEPRAPEFYFAQKIDYLKDKIQPSFVKERRAMKREYEEFKVRINALVAKAQKIPEEGWTMQDGTPWPGNNTRDHPGMIQVFLGHSGGLDTDGNELPRLIYVSREKRPGFQHHKKAGAMNALIRVSAVLTNGAYLLNVDCDHYFNNSKAIKEAMCFMMDPAIGKKCCYVQFPQRFDGIDLHDRYANRNIVFFDINMKGLDGIQGPVYVGTGCCFNRQALYGYDPVLTEEDLEPNIIVKSCCGSRKKGKSSKKYNYEKRRGINRSDSNAPLFNMEDIDEGFEGYDDERSILMSQRSVEKRFGQSPVFIAATFMEQGGIPPTTNPATLLKEAIHVISCGYEDKTEWGKEIGWIYGSVTEDILTGFKMHARGWISIYCNPPRPAFKGSAPINLSDRLNQVLRWALGSIEILLSRHCPIWYGYHGRLRLLERIAYINTIVYPITSIPLIAYCILPAFCLITDRFIIPEISNYASIWFILLFISIAVTGILELRWSGVSIEDWWRNEQFWVIGGTSAHLFAVFQGLLKVLAGIDTNFTVTSKATDEDGDFAELYIFKWTALLIPPTTVLLVNLIGIVAGVSYAVNSGYQSWDPLFGKLFFALWVIAHLYPFLKGLLGRQNRTPTIVIVWSVLLASIFSLLWVRINPFVDANPNANNFNGKGGVF

SEQ ID NO: 20 - DNA, 4690 bp, Arabidopsis thaliana
atggaatccgaaggagaaaccgcggtatgcttttttgactcttgcttcatcattatacttacctttatcgaaatcaggaattatatgtactgaaattgattgatttgggtgttgaattgtgtattggagagatctgatttcaaattttctgttgaggtttctaattttggcttcattgattcgacttgatttgtagggaaagccgatgaagaacattgttccgcagacttgccagatctgtagtgacaatgttggcaagactgttgatggagatcgttttgtggcttgtgatatttgttcattcccagtttgtcggccttgctacgagtatgagaggaaagatgggaatcaatcttgtcctcagtgcaaaaccagatacaagaggctcaaaggttctcttttgatccttctgaagtatactgtcttcattgttcatcgatagtttatcagtatgttttgaattttggatcagattggtatttatagcaatttgctaatttctgattctaggtagtcctgctattcctggtgataaagacgaggatggcttagctgatgaaggtactgttgagttcaactaccctcagaaggagaaaatttcagagcggatgcttggttggcatcttactcgtgggaagggagaggaaatgggggaaccccagtatgataaagaggtctctcacaatcatcttcctcgtctcacgagcagacaagatgtaaggcattgctgttcattcttccctcttaagcattcgcatcctcacgcaatttagttttggaatctgattttgtcatttgcttatttacagacttcaggagagttttctgctgcctcacctgaacgcctctctgtatcttctactatcgctgggggaaagcgccttccctattcatcagatgtcaatcaatcacgtaaatatcctttatttctaactctctcgccaacacatatatttgtacctaggcttctcttttatgtcaaaactctaaacaataaaatctgttgttgtcattcacgctgcagcaaatagaaggattgtggatcctgttggactcgggaatgtagcttggaaggagagagttgatggctggaaaatgaagcaagagaagaatactggtcctgtcagcacgcaggctgcttctgaaagaggtggagtagatattgatgccagcacagatatcctagcagatgaggctctgctgtgagttcttgttttgtaatcttgtttgttctgtcgtggtgtaccgagcgtttttcctattaagcaatgtcctgatactcattttccaattctttatttattgtacaggaatgacgaagcgaggcagcctctgtcaaggaaagtttcaattccttcatcacggatcaatccttacagaatggttattatgctgcggcttgttatcctttgtctcttcttgcattaccgtataacaaacccagtgccaaatgcctttgctctatggctggtctctgtgatatgtgagatctggtttgccttatcctggattttggatcagtttcccaagtggtttcctgtgaaccgtgaaacctacctcgacaggcttgctttaaggtaagttctatttccccattcttctgaagcaattactcaaaggattgtttgcctatactgtttcccattttaatttgatcatggtcaatttttgggacagatatgatcgtgaaggtgagccatcacagttagctgctgttgacattttcgtgagtactgttgaccccttgaaggagccaccccttgtgacagccaacacagtgctctctattctggctgttgactacccagttgacaaggtgtcctgttatgtttctgatgatggtgctgctatgttatcatttgaatcacttgcagaaacatcagagtttgctcgtaaatgggtaccattttgcaagaaatatagcatagagcctcgtgcaccagaatggtactttgctgcgaaaatagattacttgaaggataaagttcagacatcatttgtcaaagatcgtagagctatgaaggtaagtttgtagttttagtcatctagtcaccctcactttgattttagtgtatgctatattgaccttttattttctttcagagggaatatgaggaatttaaaatccgaatcaatgcacttgtttccaaagccctaaaatgtcctgaagaagggtgggttatgcaagatggcacaccgtggcctggaaataatacaagggaccatccaggaatgatccaggtaagaaattggttttaactatggaatcgagaatgctctctctttctctctagaagttcattattgaagtaccatttgctgaatgcaggtcttcttagggcaaaatggtggacttgatgcagagggcaatgagctcccgcgtttggtatatgtttctcgagaaaagcgaccaggattccagcaccacaaaaaggctggtgctatgaatgcactggtaagtttctgatcttggatttttgacttcttcattctgaccaatttgttagtctaatctgggtacttttcaaatgaataggtgagagtttcagcagttcttaccaatggacctttcatcttgaatcttgattgtgatcattacataaataacagcaaagccttaagagaagcaatgtgcttcctgatggacccaaacctcgggaagcaagtttgttatgttcagttcccacaaagatttgatggtatcgataagaacgatagatatgctaatcgtaataccgtgttctttgatgtaagtcacacttacctatacttgcgtctaattttcttgttctttcaaattgcttttagacacgaatatacattaaactcacagtttcttgagtttgtcgtaatttttccatgatatgttttccagattaacttgagaggtttagatgggattcaaggacctgtatatgtcggaactggatgtgttttcaacagaacagcattatacggttatgaacctccaataaaagtaaaacacaagaagccaagtcttttatctaagctctgtggtggatcaagaaagaagaattccaaagctaagaaagagtcggacaaaaagaaatcaggcaggcatactgactcaactgttcctgtattcaacctcgatgacatagaagagggagttgaaggtacaactgtttttatttcttctttggtttccgttatacccatatgttgctgtttgaaatattgatccaggggaggggattatttatagttgacagttgtctaaatagtttccatactaggtatctcatcatgtcttaactatttggcatttgtgaaacttaggtgctggttttgatgatgaaaaggcgctcttaatgtcgcaaatgagcctggagaagcgatttggacagtctgctgtttttgttgcttctaccctaatggaaaatggtggtgttcctccttcagcaactccagaaaaccttctcaaagaggctatccatgtcattagttgtggttatgaggataagtcagattggggaatggaggtataatctcatttgaactcctacatgaatctgcattgttctgacatatccactttggcattcactttgtttatattttccgctgtctttcttcagattggatggatctatggttctgtgacagaagatattctgactgggttcaaaatgcatgcccgtggatggcgatccatttactgcatgcctaagcttccagctttcaagggttctgctcctatcaatctttcagatcgtctgaaccaagtgctgaggtgggctttaggttcagttgagattctcttcagtcggcattgtcctatatggtatggttacaatgggaggctaaaatttcttgagaggtttgcgtatgtgaacaccaccatctaccctatcacctccattcctcttctcatgtattgtacattgccagccgtttgtctcttcaccaaccagtttattattcctcaggtttgacacctctctctgtctatctatctctatctctatctctatctctagaacaaaccttaattacgttctgtttaactgaaaccatgttgtgtttgtcatctatttacggttccaaatcctgatcagctggttctattgttcctcttttgcagattagtaacattgcaagtatatggtttctgtctctctttctctccattttcgccacgggtatactagaaatgaggtggagtggcgtaggcatagacgaatggtggagaaacgagcagttttgggtcattggtggagtatccgctcatttattcgctgtgtttcaaggtatcctcaaagtccttgccggtattgacacaaacttcacagttacctcaaaagcttcagatgaagacggagactttgctgagctctacttgttcaaatggacaacacttctgattccgccaacgacgctgctcattgtaaacttagtgggagttgttgcaggagtctcttatgctatcaacagtggataccaatcatggggaccactctttggtaagttgttctttgccttctgggtgattgttcacttgtaccctttcctcaagggtttgatgggtcgacagaaccggactcctaccattgttgtggtctggtctgttctcttggcttctatcttcttgttgttgtgggttaggattgatcccttcactagccgagtcactggcccggacattctggaatgtggaatcaactgttga

SEQ ID NO: 21 - protein, 1065 aa, Arabidopsis thaliana
MESEGETAGKPMKNIVPQTCQICSDNVGKTVDGDRFVACDICSFPVCRPCYEYERKDGNQSCPQCKTRYKRLKGSPAIPGDKDEDGLADEGTVEFNYPQKEKISERMLGWHLTRGKGEEMGEPQYDKEVSHNHLPRLTSRQDTSGEFSAASPERLSVSSTIAGGKRLPYSSDVNQSPNRRIVDPVGLGNVAWKERVDGWKMKQEKNTGPVSTQAASERGGVDIDASTDILADEALLNDEARQPLSRKVSIPSSRINPYRMVIMLRLVILCLFLHYRITNPVPNAFALWLVSVICEIWFALSWILDQFPKWFPVNRETYLDRLALRYDREGEPSQLAAVDIFVSTVDPLKEPPLVTANTVLSILAVDYPVDKVSCYVSDDGAAMLSFESLAETSEFARKWVPFCKKYSIEPRAPEWYFAAKIDYLKDKVQTSFVKDRRAMKREYEEFKIRINALVSKALKCPEEGWVMQDGTPWPGNNTRDHPGMIQVFLGQNGGLDAEGNELPRLVYVSREKRPGFQHHKKAGAMNALVRVSAVLTNGPFILNLDCDHYINNSKALREAMCFLMDPNLGKQVCYVQFPQRFDGIDKNDRYANRNTVFFDINLRGLDGIQGPVYVGTGCVFNRTALYGYEPPIKVKHKKPSLLSKLCGGSRKKNSKAKKESDKKKSGRHTDSTVPVFNLDDIEEGVEGAGFDDEKALLMSQMSLEKRFGQSAVFVASTLMENGGVPPSATPENLLKEAIHVISCGYEDKSDWGMEIGWIYGSVTEDILTGFKMHARGWRSIYCMPKLPAFKGSAPINLSDRLNQVLRWALGSVEILFSRHCPIWYGYNGRLKFLERFAYVNTTIYPITSIPLLMYCTLPAVCLFTNQFIIPQISNIASIWFLSLFLSIFATGILEMRWSGVGIDEWWRNEQFWVIGGVSAHLFAVFQGILKVLAGIDTNFTVTSKASDEDGDFAELYLFKWTTLLIPPTTLLIVNLVGVVAGVSYAINSGYQSWGPLFGKLFFAFWVIVHLYPFLKGLMGRQNRTPTIVVVWSVLLASIFLLLWVRIDPFTSRVTGPDILECGINC

SEQ ID NO: 22 - DNA, 4690 bp, Arabidopsis thaliana
atggaatccgaaggagaaaccgcggtatgcttttttgactcttgcttcatcattatacttacctttatcgaaatcaggaattatatgtactgaaattgattgatttgggtgttgaattgtgtattggagagatctgatttcaaattttctgttgaggtttctaattttggcttcattgattcgacttgatttgtagggaaagccgatgaagaacattgttccgcagacttgccagatctgtagtgacaatgttggcaagactgttgatggagatcgttttgtggcttgtgatatttgttcattcccagtttgtcggccttgctacgagtatgagaggaaagatgggaatcaatcttgtcctcagtgcaaaaccagatacaagaggctcaaaggttctcttttgatccttctgaagtatactgtcttcattgttcatcgatagtttatcagtatgttttgaattttggatcagattggtatttatagcaatttgctaatttctgattctaggtagtcctgctattcctggtgataaagacgaggatggcttagctgatgaaggtactgttgagttcaactaccctcagaaggagaaaatttcagagcggatgcttggttggcatcttactcgtgggaagggagaggaaatgggggaaccccagtatgataaagaggtctctcacaatcatcttcctcgtctcacgagcagacaagatgtaaggcattgctgttcattcttccctcttaagcattcgcatcctcacgcaatttagttttggaatctgattttgtcatttgcttatttacagacttcaggagagttttctgctgcctcacctgaacgcctctctgtatcttctactatcgctgggggaaagcgccttccctattcatcagatgtcaatcaatcacgtaaatatcctttatttctaactctctcgccaacacatatatttgtacctaggcttctcttttatgtcaaaactctaaacaataaaatctgttgttgtcattcacgctgcagcaaatagaaggattgtggatcctgttggactcgggaatgtagcttggaaggagagagttgatggctggaaaatgaagcaagagaagaatactggtcctgtcagcacgcaggctgcttctgaaagaggtggagtagatattgatgccagcacagatatcctagcagatgaggctctgctgtgagttcttgttttgtaatcttgtttgttctgtcgtggtgtaccgagcgtttttcctattaagcaatgtcctgatactcattttccaattctttatttattgtacaggaatgacgaagcgaggcagcctctgtcaaggaaagtttcaattccttcatcacggatcaatccttacagaatggttattatgctgcggcttgttatcctttgtctcttcttgcattaccgtataacaaacccagtgccaaatgcctttgctctatggctggtctctgtgatatgtgagatctggtttgccttatcctggattttggatcagtttcccaagtggtttcctgtgaaccgtgaaacctacctcgacaggcttgctttaaggtaagttctatttccccattcttctgaagcaattactcaaaggattgtttgcctatactgtttcccattttaatttgatcatggtcaatttttgggacagatatgatcgtgaaggtgagccatcacagttagctgctgttgacattttcgtgagtactgttgaccccttgaaggagccaccccttgtgacagccaacacagtgctctctattctggctgttgactacccagttgacaaggtgtcctgttatgtttctgatgatggtgctgctatgttatcatttgaatcacttgcagaaacatcagagtttgctcgtaaatgggtaccattttgcaagaaatatagcatagagcctcgtgcaccagaatggtactttgctgcgaaaatagattacttgaaggataaagttcagacatcatttgtcaaagatcgtagagctatgaaggtaagtttgtagttttagtcatctagtcaccctcactttgattttagtgtatgctatattgaccttttattttctttcagagggaatatgaggaatttaaaatccgaatcaatgcacttgtttccaaagccctaaaatgtcctgaagaagggtgggttatgcaagatggcacaccgtggcctggaaataatacaagggaccatccaggaatgatccaggtaagaaattggttttaactatggaatcgagaatgctctctctttctctctagaagttcattattgaagtaccatttgctgaatgcaggtcttcttagggcaaaatggtggacttgatgcagagggcaatgagctcccgcgtttggtatatgtttctcgagaaaagcgaccaggattccagcaccacaaaaaggctggtgctatgaatgcactggtaagtttctgatcttggatttttgacttcttcattctgaccaatttgttagtctaatctgggtacttttcaaatgaataggtgagagtttcagcagttcttaccaatggacctttcatcttgaatcttgattgtgatcattacataaataacagcaaagccttaagagaagcaatgtgcttcctgatggacccaaacctcgggaagcaagtttgttatgttcagttcccacaaagatttgatggtatcgataagaacgatagatatgctaatcgtaataccgtgttctttgatgtaagtcacacttacctatacttgcgtctaattttcttgttctttcaaattgcttttagacacgaatatacattaaactcacagtttcttgagtttgtcgtaatttttccatgatatgttttccagattaacttgagaggtttagatgggattcaaggacctgtatatgtcggaactggatgtgttttcaacagaacagcattatacggttatgaacctccaataaaagtaaaacacaagaagccaagtcttttatctaagctctgtggtggatcaagaaagaagaattccaaagctaagaaagagtcggacaaaaagaaatcaggcaggcatactgactcaactgttcctgtattcaacctcgatgacatagaagagggagttgaaggtacaactgtttttatttcttctttggtttccgttatacccatatgttgctgtttgaaatattgatccaggggaggggattatttatagttgacagttgtctaaatagtttccatactaggtatctcatcatgtcttaactatttggcatttgtgaaacttaggtgctggttttgatgatgaaaaggcgctcttaatgtcgcaaatgagcctggagaagcgatttggacagtctgctgtttttgttgcttctaccctaatggaaaatggtggtgttcctccttcagcaactccagaaaaccttctcaaagaggctatccatgtcattagttgtggttatgaggataagtcagattggggaatggaggtataatctcatttgaactcctacatgaatctgcattgttctgacatatccactttggcattcactttgtttatattttccgctgtctttcttcagattggatggatctatggttctgtgacagaagatattctgactgggttcaaaatgcatgcccgtggatggcgatccatttactgcatgcctaagcttccagctttcaagggttctgctcctatcaatctttcagatcgtctgaaccaagtgctgaggtgggctttaggttcagttgagattctcttcagtcggcattgtcctatatggtatggttacaatgggaggctaaaatttcttgagaggtttgcgtatgtgaacaccaccatctaccctatcacctccattcctcttctcatgtattgtacattgccagccgtttgtctcttcaccaaccagtttattattcctcaggtttgacacctctctctgtctatctatctctatctctatctctatctctagaacaaaccttaattacgttctgtttaactgaaaccatgttgtgtttgtcatctatttacggttccaaatcctgatcagctggttctattgttcctcttttgcagattagtaacattgcaagtatatggtttctgtctctctttctctccattttcgccacgggtatactagaaatgaggtggagtggcgtaggcatagacgaatggtggagaaacgagcagttttgggtcattggtggagtatccgctcatttattcgctgtgtttcaaggtatcctcaaagtccttgccggtattgacacaaacttcacagttacctcaaaagcttcagatgaagacggagactttgctgagctctacttgttcaaatggacaacacttctgattccgccaacgacgctgctcattgtaaacttagtgggagttgttgcaggagtctcttatgctatcaacagtggataccaatcatggggaccactctttggtaagttgttctttgccttctgggtgattgttcacttgtaccctttcctcaagggtttgatgggtcgacagaaccggactcctaccattgttgtggtctggtctgttctcttggcttttatcttctcgttgttgtgggttaggattgatcccttcactagccgagtcactggcccggacattctggaatgtggaatcaactgttga

SEQ ID NO: 23 - protein, 1065 aa, Arabidopsis thaliana
MESEGETAGKPMKNIVPQTCQICSDNVGKTVDGDRFVACDICSFPVCRPCYEYERKDGNQSCPQCKTRYKRLKGSPAIPGDKDEDGLADEGTVEFNYPQKEKISERMLGWHLTRGKGEEMGEPQYDKEVSHNHLPRLTSRQDTSGEFSAASPERLSVSSTIAGGKRLPYSSDVNQSPNRRIVDPVGLGNVAWKERVDGWKMKQEKNTGPVSTQAASERGGVDIDASTDILADEALLNDEARQPLSRKVSIPSSRINPYRMVIMLRLVILCLFLHYRITNPVPNAFALWLVSVICEIWFALSWILDQFPKWFPVNRETYLDRLALRYDREGEPSQLAAVDIFVSTVDPLKEPPLVTANTVLSILAVDYPVDKVSCYVSDDGAAMLSFESLAETSEFARKWVPFCKKYSIEPRAPEWYFAAKIDYLKDKVQTSFVKDRRAMKREYEEFKIRINALVSKALKCPEEGWVMQDGTPWPGNNTRDHPGMIQVFLGQNGGLDAEGNELPRLVYVSREKRPGFQHHKKAGAMNALVRVSAVLTNGPFILNLDCDHYINNSKALREAMCFLMDPNLGKQVCYVQFPQRFDGIDKNDRYANRNTVFFDINLRGLDGIQGPVYVGTGCVFNRTALYGYEPPIKVKHKKPSLLSKLCGGSRKKNSKAKKESDKKKSGRHTDSTVPVFNLDDIEEGVEGAGFDDEKALLMSQMSLEKRFGQSAVFVASTLMENGGVPPSATPENLLKEAIHVISCGYEDKSDWGMEIGWIYGSVTEDILTGFKMHARGWRSIYCMPKLPAFKGSAPINLSDRLNQVLRWALGSVEILFSRHCPIWYGYNGRLKFLERFAYVNTTIYPITSIPLLMYCTLPAVCLFTNQFIIPQISNIASIWFLSLFLSIFATGILEMRWSGVGIDEWWRNEQFWVIGGVSAHLFAVFQGILKVLAGIDTNFTVTSKASDEDGDFAELYLFKWTTLLIPPTTLLIVNLVGVVAGVSYAINSGYQSWGPLFGKLFFAFWVIVHLYPFLKGLMGRQNRTPTIVVVWSVLLAFIFSLLWVRIDPFTSRVTGPDILECGINC

SEQ ID NO: 24 - DNA, 4690 bp, Arabidopsis thaliana
atggaatccgaaggagaaaccgcggtatgcttttttgactcttgcttcatcattatacttacctttatcgaaatcaggaattatatgtactgaaattgattgatttgggtgttgaattgtgtattggagagatctgatttcaaattttctgttgaggtttctaattttggcttcattgattcgacttgatttgtagggaaagccgatgaagaacattgttccgcagacttgccagatctgtagtgacaatgttggcaagactgttgatggagatcgttttgtggcttgtgatatttgttcattcccagtttgtcggccttgctacgagtatgagaggaaagatgggaatcaatcttgtcctcagtgcaaaaccagatacaagaggctcaaaggttctcttttgatccttctgaagtatactgtcttcattgttcatcgatagtttatcagtatgttttgaattttggatcagattggtatttatagcaatttgctaatttctgattctaggtagtcctgctattcctggtgataaagacgaggatggcttagctgatgaaggtactgttgagttcaactaccctcagaaggagaaaatttcagagcggatgcttggttggcatcttactcgtgggaagggagaggaaatgggggaaccccagtatgataaagaggtctctcacaatcatcttcctcgtctcacgagcagacaagatgtaaggcattgctgttcattcttccctcttaagcattcgcatcctcacgcaatttagttttggaatctgattttgtcatttgcttatttacagacttcaggagagttttctgctgcctcacctgaacgcctctctgtatcttctactatcgctgggggaaagcgccttccctattcatcagatgtcaatcaatcacgtaaatatcctttatttctaactctctcgccaacacatatatttgtacctaggcttctcttttatgtcaaaactctaaacaataaaatctgttgttgtcattcacgctgcagcaaatagaaggattgtggatcctgttggactcgggaatgtagcttggaaggagagagttgatggctggaaaatgaagcaagagaagaatactggtcctgtcagcacgcaggctgcttctgaaagaggtggagtagatattgatgccagcacagatatcctagcagatgaggctctgctgtgagttcttgttttgtaatcttgtttgttctgtcgtggtgtaccgagcgtttttcctattaagcaatgtcctgatactcattttccaattctttatttattgtacaggaatgacgaagcgaggcagcctctgtcaaggaaagtttcaattccttcatcacggatcaatccttacagaatggttattatgctgcggcttgttatcctttgtctcttcttgcattaccgtataacaaacccagtgccaaatgcctttgctctatggctggtctctgtgatatgtgagatctggtttgccttatcctggattttggatcagtttcccaagtggtttcctgtgaaccgtgaaacctacctcgacaggcttgctttaaggtaagttctatttccccattcttctgaagcaattactcaaaggattgtttgcctatactgtttcccattttaatttgatcatggtcaatttttgggacagatatgatcgtgaaggtgagccatcacagttagctgctgttgacattttcgtgagtactgttgaccccttgaaggagccaccccttgtgacagccaacacagtgctctctattctggctgttgactacccagttgacaaggtgtcctgttatgtttctgatgatggtgctgctatgttatcatttgaatcacttgcagaaacatcagagtttgctcgtaaatgggtaccattttgcaagaaatatagcatagagcctcgtgcaccagaatggtactttgctgcgaaaatagattacttgaaggataaagttcagacatcatttgtcaaagatcgtagagctatgaaggtaagtttgtagttttagtcatctagtcaccctcactttgattttagtgtatgctatattgaccttttattttctttcagagggaatatgaggaatttaaaatccgaatcaatgcacttgtttccaaagccctaaaatgtcctgaagaagggtgggttatgcaagatggcacaccgtggcctggaaataatacaagggaccatccaggaatgatccaggtaagaaattggttttaactatggaatcgagaatgctctctctttctctctagaagttcattattgaagtaccatttgctgaatgcaggtcttcttagggcaaaatggtggacttgatgcagagggcaatgagctcccgcgtttggtatatgtttctcgagaaaagcgaccaggattccagcaccacaaaaaggctggtgctatgaatgcactggtaagtttctgatcttggatttttgacttcttcattctgaccaatttgttagtctaatctgggtacttttcaaatgaataggtgagagtttcagcagttcttaccaatggacctttcatcttgaatcttgattgtgatcattacataaataacagcaaagccttaagagaagcaatgtgcttcctgatggacccaaacctcgggaagcaagtttgttatgttcagttcccacaaagatttgatggtatcgataagaacgatagatatgctaatcgtaataccgtgttctttgatgtaagtcacacttacctatacttgcgtctaattttcttgttctttcaaattgcttttagacacgaatatacattaaactcacagtttcttgagtttgtcgtaatttttccatgatatgttttccagattaacttgagaggtttagatgggattcaaggacctgtatatgtcggaactggatgtgttttcaacagaacagcattatacggttatgaacctccaataaaagtaaaacacaagaagccaagtcttttatctaagctctgtggtggatcaagaaagaagaattccaaagctaagaaagagtcggacaaaaagaaatcaggcaggcatactgactcaactgttcctgtattcaacctcgatgacatagaagagggagttgaaggtacaactgtttttatttcttctttggtttccgttatacccatatgttgctgtttgaaatattgatccaggggaggggattatttatagttgacagttgtctaaatagtttccatactaggtatctcatcatgtcttaactatttggcatttgtgaaacttaggtgctggttttgatgatgaaaaggcgctcttaatgtcgcaaatgagcctggagaagcgatttggacagtctgctgtttttgttgcttctaccctaatggaaaatggtggtgttcctccttcagcaactccagaaaaccttctcaaagaggctatccatgtcattagttgtggttatgaggataagtcagattggggaatggaggtataatctcatttgaactcctacatgaatctgcattgttctgacatatccactttggcattcactttgtttatattttccgctgtctttcttcagattggatggatctatggttctgtgacagaagatattctgactgggttcaaaatgcatgcccgtggatggcgatccatttactgcatgcctaagcttccagctttcaagggttctgctcctatcaatctttcagatcgtctgaaccaagtgctgaggtgggctttaggttcagttgagattctcttcagtcggcattgtcctatatggtatggttacaatgggaggctaaaatttcttgagaggtttgcgtatgtgaacaccaccatctaccctatcacctccattcctcttctcatgtattgtacattgccagccgtttgtctcttcaccaaccagtttattattcctcaggtttgacacctctctctgtctatctatctctatctctatctctatctctagaacaaaccttaattacgttctgtttaactgaaaccatgttgtgtttgtcatctatttacggttccaaatcctgatcagctggttctattgttcctcttttgcagattagtaacattgcaagtatatggtttctgtctctctttctctccattttcgccacgggtatactagaaatgaggtggagtggcgtaggcatagacgaatggtggagaaacgagcagttttgggtcattggtggagtatccgctcatttattcgctgtgtttcaaggtatcctcaaagtccttgccggtattgacacaaacttcacagttacctcaaaagcttcagatgaagacggagactttgctgagctctacttgttcaaatggacaacacttctgattccgccaacgacgctgctcattgtaaacttagtgggagttgttgcaggagtcttttatgctatcaacagtggataccaatcatggggaccactctttggtaagttgttctttgccttctgggtgattgttcacttgtaccctttcctcaagggtttgatgggtcgacagaaccggactcctaccattgttgtggtctggtctgttctcttggcttctatcttctcgttgttgtgggttaggattgatcccttcactagccgagtcactggcccggacattctggaatgtggaatcaactgttga

SEQ ID NO: 25 - protein, 1065 aa, Arabidopsis thaliana
MESEGETAGKPMKNIVPQTCQICSDNVGKTVDGDRFVACDICSFPVCRPCYEYERKDGNQSCPQCKTRYKRLKGSPAIPGDKDEDGLADEGTVEFNYPQKEKISERMLGWHLTRGKGEEMGEPQYDKEVSHNHLPRLTSRQDTSGEFSAASPERLSVSSTIAGGKRLPYSSDVNQSPNRRIVDPVGLGNVAWKERVDGWKMKQEKNTGPVSTQAASERGGVDIDASTDILADEALLNDEARQPLSRKVSIPSSRINPYRMVIMLRLVILCLFLHYRITNPVPNAFALWLVSVICEIWFALSWILDQFPKWFPVNRETYLDRLALRYDREGEPSQLAAVDIFVSTVDPLKEPPLVTANTVLSILAVDYPVDKVSCYVSDDGAAMLSFESLAETSEFARKWVPFCKKYSIEPRAPEWYFAAKIDYLKDKVQTSFVKDRRAMKREYEEFKIRINALVSKALKCPEEGWVMQDGTPWPGNNTRDHPGMIQVFLGQNGGLDAEGNELPRLVYVSREKRPGFQHHKKAGAMNALVRVSAVLTNGPFILNLDCDHYINNSKALREAMCFLMDPNLGKQVCYVQFPQRFDGIDKNDRYANRNTVFFDINLRGLDGIQGPVYVGTGCVFNRTALYGYEPPIKVKHKKPSLLSKLCGGSRKKNSKAKKESDKKKSGRHTDSTVPVFNLDDIEEGVEGAGFDDEKALLMSQMSLEKRFGQSAVFVASTLMENGGVPPSATPENLLKEAIHVISCGYEDKSDWGMEIGWIYGSVTEDILTGFKMHARGWRSIYCMPKLPAFKGSAPINLSDRLNQVLRWALGSVEILFSRHCPIWYGYNGRLKFLERFAYVNTTIYPITSIPLLMYCTLPAVCLFTNQFIIPQISNIASIWFLSLFLSIFATGILEMRWSGVGIDEWWRNEQFWVIGGVSAHLFAVFQGILKVLAGIDTNFTVTSKASDEDGDFAELYLFKWTTLLIPPTTLLIVNLVGVVAGVFYAINSGYQSWGPLFGKLFFAFWVIVHLYPFLKGLMGRQNRTPTIVVVWSVLLASIFSLLWVRIDPFTSRVTGPDILECGINC

SEQ ID NO: 26 - DNA, 4690 bp, Arabidopsis thaliana
atggaatccgaaggagaaaccgcggtatgcttttttgactcttgcttcatcattatacttacctttatcgaaatcaggaattatatgtactgaaattgattgatttgggtgttgaattgtgtattggagagatctgatttcaaattttctgttgaggtttctaattttggcttcattgattcgacttgatttgtagggaaagccgatgaagaacattgttccgcagacttgccagatctgtagtgacaatgttggcaagactgttgatggagatcgttttgtggcttgtgatatttgttcattcccagtttgtcggccttgctacgagtatgagaggaaagatgggaatcaatcttgtcctcagtgcaaaaccagatacaagaggctcaaaggttctcttttgatccttctgaagtatactgtcttcattgttcatcgatagtttatcagtatgttttgaattttggatcagattggtatttatagcaatttgctaatttctgattctaggtagtcctgctattcctggtgataaagacgaggatggcttagctgatgaaggtactgttgagttcaactaccctcagaaggagaaaatttcagagcggatgcttggttggcatcttactcgtgggaagggagaggaaatgggggaaccccagtatgataaagaggtctctcacaatcatcttcctcgtctcacgagcagacaagatgtaaggcattgctgttcattcttccctcttaagcattcgcatcctcacgcaatttagttttggaatctgattttgtcatttgcttatttacagacttcaggagagttttctgctgcctcacctgaacgcctctctgtatcttctactatcgctgggggaaagcgccttccctattcatcagatgtcaatcaatcacgtaaatatcctttatttctaactctctcgccaacacatatatttgtacctaggcttctcttttatgtcaaaactctaaacaataaaatctgttgttgtcattcacgctgcagcaaatagaaggattgtggatcctgttggactcgggaatgtagcttggaaggagagagttgatggctggaaaatgaagcaagagaagaatactggtcctgtcagcacgcaggctgcttctgaaagaggtggagtagatattgatgccagcacagatatcctagcagatgaggctctgctgtgagttcttgttttgtaatcttgtttgttctgtcgtggtgtaccgagcgtttttcctattaagcaatgtcctgatactcattttccaattctttatttattgtacaggaatgacgaagcgaggcagcctctgtcaaggaaagtttcaattccttcatcacggatcaatccttacagaatggttattatgctgcggcttgttatcctttgtctcttcttgcattaccgtataacaaacccagtgccaaatgcctttgctctatggctggtctctgtgatatgtgagatctggtttgccttatcctggattttggatcagtttcccaagtggtttcctgtgaaccgtgaaacctacctcgacaggcttgctttaaggtaagttctatttccccattcttctgaagcaattactcaaaggattgtttgcctatactgtttcccattttaatttgatcatggtcaatttttgggacagatatgatcgtgaaggtgagccatcacagttagctgctgttgacattttcgtgagtactgttgaccccttgaaggagccaccccttgtgacagccaacacagtgctctctattctggctgttgactacccagttgacaaggtgtcctgttatgtttctgatgatggtgctgctatgttatcatttgaatcacttgcagaaacatcagagtttgctcgtaaatgggtaccattttgcaagaaatatagcatagagcctcgtgcaccagaatggtactttgctgcgaaaatagattacttgaaggataaagttcagacatcatttgtcaaagatcgtagagctatgaaggtaagtttgtagttttagtcatctagtcaccctcactttgattttagtgtatgctatattgaccttttattttctttcagagggaatatgaggaatttaaaatccgaatcaatgcacttgtttccaaagccctaaaatgtcctgaagaagggtgggttatgcaagatggcacaccgtggcctggaaataatacaagggaccatccaggaatgatccaggtaagaaattggttttaactatggaatcgagaatgctctctctttctctctagaagttcattattgaagtaccatttgctgaatgcaggtcttcttagggcaaaatggtggacttgatgcagagggcaatgagctcccgcgtttggtatatgtttctcgagaaaagcgaccaggattccagcaccacaaaaaggctggtgctatgaatgcactggtaagtttctgatcttggatttttgacttcttcattctgaccaatttgttagtctaatctgggtacttttcaaatgaataggtgagagtttcagcagttcttaccaatggacctttcatcttgaatcttgattgtgatcattacataaataacagcaaagccttaagagaagcaatgtgcttcctgatggacccaaacctcgggaagcaagtttgttatgttcagttcccacaaagatttgatggtatcgataagaacgatagatatgctaatcgtaataccgtgttctttgatgtaagtcacacttacctatacttgcgtctaattttcttgttctttcaaattgcttttagacacgaatatacattaaactcacagtttcttgagtttgtcgtaatttttccatgatatgttttccagattaacttgagaggtttagatgggattcaaggacctgtatatgtcggaactggatgtgttttcaacagaacagcattatacggttatgaacctccaataaaagtaaaacacaagaagccaagtcttttatctaagctctgtggtggatcaagaaagaagaattccaaagctaagaaagagtcggacaaaaagaaatcaggcaggcatactgactcaactgttcctgtattcaacctcgatgacatagaagagggagttgaaggtacaactgtttttatttcttctttggtttccgttatacccatatgttgctgtttgaaatattgatccaggggaggggattatttatagttgacagttgtctaaatagtttccatactaggtatctcatcatgtcttaactatttggcatttgtgaaacttaggtgctggttttgatgatgaaaaggcgctcttaatgtcgcaaatgagcctggagaagcgatttggacagtctgctgtttttgttgcttctaccctaatggaaaatggtggtgttcctccttcagcaactccagaaaaccttctcaaagaggctatccatgtcattagttgtggttatgaggataagtcagattggggaatggaggtataatctcatttgaactcctacatgaatctgcattgttctgacatatccactttggcattcactttgtttatattttccgctgtctttcttcagattggatggatctatggttctgtgacagaagatattctgactgggttcaaaatgcatgcccgtggatggcgatccatttactgcatgcctaagcttccagctttcaagggttctgctcctatcaatctttcagatcgtctgaaccaagtgctgaggtgggctttaggttcagttgagattctcttcagtcggcattgtcctatatggtatggttacaatgggaggctaaaatttcttgagaggtttgcgtatgtgaacaccaccatctaccctatcacctccattcctcttctcatgtattgtacattgccagccgtttgtctcttcaccaaccagtttattattcctcaggtttgacacctctctctgtctatctatctctatctctatctctatctctagaacaaaccttaattacgttctgtttaactgaaaccatgttgtgtttgtcatctatttacggttccaaatcctgatcagctggttctattgttcctcttttgcagattagtaacattgcaagtatatggtttctgtctctctttctctccattttcgccacgggtatactagaaatgaggtggagtggcgtaggcatagacgaatggtggagaaacgagcagttttgggtcattggtggagtatccgctcatttattcgctgtgtttcaaggtatcctcaaagtccttgccggtattgacacaaacttcacagttacctcaaaagcttcagatgaagacggagactttgctgagctctacttgttcaaatggacaacacttctgattccgccaacgacgctgctcattgtaaacttagtgggagttgttgcaggagtctcttatgctatcaacagtggataccaatcatggggaccactctttagtaagttgttctttgccttctgggtgattgttcacttgtaccctttcctcaagggtttgatgggtcgacagaaccggactcctaccattgttgtggtctggtctgttctcttggcttctatcttctcgttgttgtgggttaggattgatcccttcactagccgagtcactggcccggacattctggaatgtggaatcaactgttga

SEQ ID NO: 27 - protein, 1065 aa, Arabidopsis thaliana
MESEGETAGKPMKNIVPQTCQICSDNVGKTVDGDRFVACDICSFPVCRPCYEYERKDGNQSCPQCKTRYKRLKGSPAIPGDKDEDGLADEGTVEFNYPQKEKISERMLGWHLTRGKGEEMGEPQYDKEVSHNHLPRLTSRQDTSGEFSAASPERLSVSSTIAGGKRLPYSSDVNQSPNRRIVDPVGLGNVAWKERVDGWKMKQEKNTGPVSTQAASERGGVDIDASTDILADEALLNDEARQPLSRKVSIPSSRINPYRMVIMLRLVILCLFLHYRITNPVPNAFALWLVSVICEIWFALSWILDQFPKWFPVNRETYLDRLALRYDREGEPSQLAAVDIFVSTVDPLKEPPLVTANTVLSILAVDYPVDKVSCYVSDDGAAMLSFESLAETSEFARKWVPFCKKYSIEPRAPEWYFAAKIDYLKDKVQTSFVKDRRAMKREYEEFKIRINALVSKALKCPEEGWVMQDGTPWPGNNTRDHPGMIQVFLGQNGGLDAEGNELPRLVYVSREKRPGFQHHKKAGAMNALVRVSAVLTNGPFILNLDCDHYINNSKALREAMCFLMDPNLGKQVCYVQFPQRFDGIDKNDRYANRNTVFFDINLRGLDGIQGPVYVGTGCVFNRTALYGYEPPIKVKHKKPSLLSKLCGGSRKKNSKAKKESDKKKSGRHTDSTVPVFNLDDIEEGVEGAGFDDEKALLMSQMSLEKRFGQSAVFVASTLMENGGVPPSATPENLLKEAIHVISCGYEDKSDWGMEIGWIYGSVTEDILTGFKMHARGWRSIYCMPKLPAFKGSAPINLSDRLNQVLRWALGSVEILFSRHCPIWYGYNGRLKFLERFAYVNTTIYPITSIPLLMYCTLPAVCLFTNQFIIPQISNIASIWFLSLFLSIFATGILEMRWSGVGIDEWWRNEQFWVIGGVSAHLFAVFQGILKVLAGIDTNFTVTSKASDEDGDFAELYLFKWTTLLIPPTTLLIVNLVGVVAGVSYAINSGYQSWGPLFSKLFFAFWVIVHLYPFLKGLMGRQNRTPTIVVVWSVLLASIFSLLWVRIDPFTSRVTGPDILECGINC

SEQ ID NO: 28 - DNA, 4690 bp, Arabidopsis thaliana
atggaatccgaaggagaaaccgcggtatgcttttttgactcttgcttcatcattatacttacctttatcgaaatcaggaattatatgtactgaaattgattgatttgggtgttgaattgtgtattggagagatctgatttcaaattttctgttgaggtttctaattttggcttcattgattcgacttgatttgtagggaaagccgatgaagaacattgttccgcagacttgccagatctgtagtgacaatgttggcaagactgttgatggagatcgttttgtggcttgtgatatttgttcattcccagtttgtcggccttgctacgagtatgagaggaaagatgggaatcaatcttgtcctcagtgcaaaaccagatacaagaggctcaaaggttctcttttgatccttctgaagtatactgtcttcattgttcatcgatagtttatcagtatgttttgaattttggatcagattggtatttatagcaatttgctaatttctgattctaggtagtcctgctattcctggtgataaagacgaggatggcttagctgatgaaggtactgttgagttcaactaccctcagaaggagaaaatttcagagcggatgcttggttggcatcttactcgtgggaagggagaggaaatgggggaaccccagtatgataaagaggtctctcacaatcatcttcctcgtctcacgagcagacaagatgtaaggcattgctgttcattcttccctcttaagcattcgcatcctcacgcaatttagttttggaatctgattttgtcatttgcttatttacagacttcaggagagttttctgctgcctcacctgaacgcctctctgtatcttctactatcgctgggggaaagcgccttccctattcatcagatgtcaatcaatcacgtaaatatcctttatttctaactctctcgccaacacatatatttgtacctaggcttctcttttatgtcaaaactctaaacaataaaatctgttgttgtcattcacgctgcagcaaatagaaggattgtggatcctgttggactcgggaatgtagcttggaaggagagagttgatggctggaaaatgaagcaagagaagaatactggtcctgtcagcacgcaggctgcttctgaaagaggtggagtagatattgatgccagcacagatatcctagcagatgaggctctgctgtgagttcttgttttgtaatcttgtttgttctgtcgtggtgtaccgagcgtttttcctattaagcaatgtcctgatactcattttccaattctttatttattgtacaggaatgacgaagcgaggcagcctctgtcaaggaaagtttcaattccttcatcacggatcaatccttacagaatggttattatgctgcggcttgttatcctttgtctcttcttgcattaccgtataacaaacccagtgccaaatgcctttgctctatggctggtctctgtgatatgtgagatctggtttgccttatcctggattttggatcagtttcccaagtggtttcctgtgaaccgtgaaacctacctcgacaggcttgctttaaggtaagttctatttccccattcttctgaagcaattactcaaaggattgtttgcctatactgtttcccattttaatttgatcatggtcaatttttgggacagatatgatcgtgaaggtgagccatcacagttagctgctgttgacattttcgtgagtactgttgaccccttgaaggagccaccccttgtgacagccaacacagtgctctctattctggctgttgactacccagttgacaaggtgtcctgttatgtttctgatgatggtgctgctatgttatcatttgaatcacttgcagaaacatcagagtttgctcgtaaatgggtaccattttgcaagaaatatagcatagagcctcgtgcaccagaatggtactttgctgcgaaaatagattacttgaaggataaagttcagacatcatttgtcaaagatcgtagagctatgaaggtaagtttgtagttttagtcatctagtcaccctcactttgattttagtgtatgctatattgaccttttattttctttcagagggaatatgaggaatttaaaatccgaatcaatgcacttgtttccaaagccctaaaatgtcctgaagaagggtgggttatgcaagatggcacaccgtggcctggaaataatacaagggaccatccaggaatgatccaggtaagaaattggttttaactatggaatcgagaatgctctctctttctctctagaagttcattattgaagtaccatttgctgaatgcaggtcttcttagggcaaaatggtggacttgatgcagagggcaatgagctcccgcgtttggtatatgtttctcgagaaaagcgaccaggattccagcaccacaaaaaggctggtgctatgaatgcactggtaagtttctgatcttggatttttgacttcttcattctgaccaatttgttagtctaatctgggtacttttcaaatgaataggtgagagtttcagcagttcttaccaatggacctttcatcttgaatcttgattgtgatcattacataaataacagcaaagccttaagagaagcaatgtgcttcctgatggacccaaacctcgggaagcaagtttgttatgttcagttcccacaaagatttgatggtatcgataagaacgatagatatgctaatcgtaataccgtgttctttgatgtaagtcacacttacctatacttgcgtctaattttcttgttctttcaaattgcttttagacacgaatatacattaaactcacagtttcttgagtttgtcgtaatttttccatgatatgttttccagattaacttgagaggtttagatgggattcaaggacctgtatatgtcggaactggatgtgttttcaacagaacagcattatacggttatgaacctccaataaaagtaaaacacaagaagccaagtcttttatctaagctctgtggtggatcaagaaagaagaattccaaagctaagaaagagtcggacaaaaagaaatcaggcaggcatactgactcaactgttcctgtattcaacctcgatgacatagaagagggagttgaaggtacaactgtttttatttcttctttggtttccgttatacccatatgttgctgtttgaaatattgatccaggggaggggattatttatagttgacagttgtctaaatagtttccatactaggtatctcatcatgtcttaactatttggcatttgtgaaacttaggtgctggttttgatgatgaaaaggcgctcttaatgtcgcaaatgagcctggagaagcgatttggacagtctgctgtttttgttgcttctaccctaatggaaaatggtggtgttcctccttcagcaactccagaaaaccttctcaaagaggctatccatgtcattagttgtggttatgaggataagtcagattggggaatggaggtataatctcatttgaactcctacatgaatctgcattgttctgacatatccactttggcattcactttgtttatattttccgctgtctttcttcagattggatggatctatggttctgtgacagaagatattctgactgggttcaaaatgcatgcccgtggatggcgatccatttactgcatgcctaagcttccagctttcaagggttctgctcctatcaatctttcagatcgtctgaaccaagtgctgaagtgggctttaggttcagttgagattctcttcagtcggcattgtcctatatggtatggttacaatgggaggctaaaatttcttgagaggtttgcgtatgtgaacaccaccatctaccctatcacctccattcctcttctcatgtattgtacattgccagccgtttgtctcttcaccaaccagtttattattcctcaggtttgacacctctctctgtctatctatctctatctctatctctatctctagaacaaaccttaattacgttctgtttaactgaaaccatgttgtgtttgtcatctatttacggttccaaatcctgatcagctggttctattgttcctcttttgcagattagtaacattgcaagtatatggtttctgtctctctttctctccattttcgccacgggtatactagaaatgaggtggagtggcgtaggcatagacgaatggtggagaaacgagcagttttgggtcattggtggagtatccgctcatttattcgctgtgtttcaaggtatcctcaaagtccttgccggtattgacacaaacttcacagttacctcaaaagcttcagatgaagacggagactttgctgagctctacttgttcaaatggacaacacttctgattccgccaacgacgctgctcattgtaaacttagtgggagttgttgcaggagtctcttatgctatcaacagtggataccaatcatggggaccactctttggtaagttgttctttgccttctgggtgattgttcacttgtaccctttcctcaagggtttgatgggtcgacagaaccggactcctaccattgttgtggtctggtctgttctcttggcttctatcttctcgttgttgtgggttaggattgatcccttcactagccgagtcactggcccggacattctggaatgtggaatcaactgttga

SEQ ID NO: 29 - protein, 1065 aa, Arabidopsis thaliana
MESEGETAGKPMKNIVPQTCQICSDNVGKTVDGDRFVACDICSFPVCRPCYEYERKDGNQSCPQCKTRYKRLKGSPAIPGDKDEDGLADEGTVEFNYPQKEKISERMLGWHLTRGKGEEMGEPQYDKEVSHNHLPRLTSRQDTSGEFSAASPERLSVSSTIAGGKRLPYSSDVNQSPNRRIVDPVGLGNVAWKERVDGWKMKQEKNTGPVSTQAASERGGVDIDASTDILADEALLNDEARQPLSRKVSIPSSRINPYRMVIMLRLVILCLFLHYRITNPVPNAFALWLVSVICEIWFALSWILDQFPKWFPVNRETYLDRLALRYDREGEPSQLAAVDIFVSTVDPLKEPPLVTANTVLSILAVDYPVDKVSCYVSDDGAAMLSFESLAETSEFARKWVPFCKKYSIEPRAPEWYFAAKIDYLKDKVQTSFVKDRRAMKREYEEFKIRINALVSKALKCPEEGWVMQDGTPWPGNNTRDHPGMIQVFLGQNGGLDAEGNELPRLVYVSREKRPGFQHHKKAGAMNALVRVSAVLTNGPFILNLDCDHYINNSKALREAMCFLMDPNLGKQVCYVQFPQRFDGIDKNDRYANRNTVFFDINLRGLDGIQGPVYVGTGCVFNRTALYGYEPPIKVKHKKPSLLSKLCGGSRKKNSKAKKESDKKKSGRHTDSTVPVFNLDDIEEGVEGAGFDDEKALLMSQMSLEKRFGQSAVFVASTLMENGGVPPSATPENLLKEAIHVISCGYEDKSDWGMEIGWIYGSVTEDILTGFKMHARGWRSIYCMPKLPAFKGSAPINLSDRLNQVLKWALGSVEILFSRHCPIWYGYNGRLKFLERFAYVNTTIYPITSIPLLMYCTLPAVCLFTNQFIIPQISNIASIWFLSLFLSIFATGILEMRWSGVGIDEWWRNEQFWVIGGVSAHLFAVFQGILKVLAGIDTNFTVTSKASDEDGDFAELYLFKWTTLLIPPTTLLIVNLVGVVAGVSYAINSGYQSWGPLFGKLFFAFWVIVHLYPFLKGLMGRQNRTPTIVVVWSVLLASIFSLLWVRIDPFTSRVTGPDILECGINC

SEQ ID NO: 30 - DNA, 4690 bp, Arabidopsis thaliana
atggaatccgaaggagaaaccgcggtatgcttttttgactcttgcttcatcattatacttacctttatcgaaatcaggaattatatgtactgaaattgattgatttgggtgttgaattgtgtattggagagatctgatttcaaattttctgttgaggtttctaattttggcttcattgattcgacttgatttgtagggaaagccgatgaagaacattgttccgcagacttgccagatctgtagtgacaatgttggcaagactgttgatggagatcgttttgtggcttgtgatatttgttcattcccagtttgtcggccttgctacgagtatgagaggaaagatgggaatcaatcttgtcctcagtgcaaaaccagatacaagaggctcaaaggttctcttttgatccttctgaagtatactgtcttcattgttcatcgatagtttatcagtatgttttgaattttggatcagattggtatttatagcaatttgctaatttctgattctaggtagtcctgctattcctggtgataaagacgaggatggcttagctgatgaaggtactgttgagttcaactaccctcagaaggagaaaatttcagagcggatgcttggttggcatcttactcgtgggaagggagaggaaatgggggaaccccagtatgataaagaggtctctcacaatcatcttcctcgtctcacgagcagacaagatgtaaggcattgctgttcattcttccctcttaagcattcgcatcctcacgcaatttagttttggaatctgattttgtcatttgcttatttacagacttcaggagagttttctgctgcctcacctgaacgcctctctgtatcttctactatcgctgggggaaagcgccttccctattcatcagatgtcaatcaatcacgtaaatatcctttatttctaactctctcgccaacacatatatttgtacctaggcttctcttttatgtcaaaactctaaacaataaaatctgttgttgtcattcacgctgcagcaaatagaaggattgtggatcctgttggactcgggaatgtagcttggaaggagagagttgatggctggaaaatgaagcaagagaagaatactggtcctgtcagcacgcaggctgcttctgaaagaggtggagtagatattgatgccagcacagatatcctagcagatgaggctctgctgtgagttcttgttttgtaatcttgtttgttctgtcgtggtgtaccgagcgtttttcctattaagcaatgtcctgatactcattttccaattctttatttattgtacaggaatgacgaagcgaggcagcctctgtcaaggaaagtttcaattccttcatcacggatcaatccttacagaatggttattatgctgcggcttgttatcctttgtctcttcttgcattaccgtataacaaacccagtgccaaatgcctttgctctatggctggtctctgtgatatgtgagatctggtttgccttatcctggattttggatcagtttcccaagtggtttcctgtgaaccgtgaaacctacctcgacaggcttgctttaaggtaagttctatttccccattcttctgaagcaattactcaaaggattgtttgcctatactgtttcccattttaatttgatcatggtcaatttttgggacagatatgatcgtgaaggtgagccatcacagttagctgctgttgacattttcgtgagtactgttgaccccttgaaggagccaccccttgtgacagccaacacagtgctctctattctggctgttgactacccagttgacaaggtgtcctgttatgtttctgatgatggtgctgctatgttatcatttgaatcacttgcagaaacatcagagtttgctcgtaaatgggtaccattttgcaagaaatatagcatagagcctcgtgcaccagaatggtactttgctgcgaaaatagattacttgaaggataaagttcagacatcatttgtcaaagatcgtagagctatgaaggtaagtttgtagttttagtcatctagtcaccctcactttgattttagtgtatgctatattgaccttttattttctttcagagggaatatgaggaatttaaaatccgaatcaatgcacttgtttccaaagccctaaaatgtcctgaagaagggtgggttatgcaagatggcacaccgtggcctggaaataatacaagggaccatccaggaatgatccaggtaagaaattggttttaactatggaatcgagaatgctctctctttctctctagaagttcattattgaagtaccatttgctgaatgcaggtcttcttagggcaaaatggtggacttgatgcagagggcaatgagctcccgcgtttggtatatgtttctcgagaaaagcgaccaggattccagcaccacaaaaaggctggtgctatgaatgcactggtaagtttctgatcttggatttttgacttcttcattctgaccaatttgttagtctaatctgggtacttttcaaatgaataggtgagagtttcagcagttcttaccaatggacctttcatcttgaatcttgattgtgatcattacataaataacagcaaagccttaagagaagcaatgtgcttcctgatggacccaaacctcgggaagcaagtttgttatgttcagttcccacaaagatttgatggtatcgataagaacgatagatatgctaatcgtaataccgtgttctttgatgtaagtcacacttacctatacttgcgtctaattttcttgttctttcaaattgcttttagacacgaatatacattaaactcacagtttcttgagtttgtcgtaatttttccatgatatgttttccagattaacttgagaggtttagatgggattcaaggacctgtatatgtcggaactggatgtgttttcaacagaacagcattatacggttatgaacctccaataaaagtaaaacacaagaagccaagtcttttatctaagctctgtggtggatcaagaaagaagaattccaaagctaagaaagagtcggacaaaaagaaatcaggcaggcatactgactcaactgttcctgtattcaacctcgatgacatagaagagggagttgaaggtacaactgtttttatttcttctttggtttccgttatacccatatgttgctgtttgaaatattgatccaggggaggggattatttatagttgacagttgtctaaatagtttccatactaggtatctcatcatgtcttaactatttggcatttgtgaaacttaggtgctggttttgatgatgaaaaggcgctcttaatgtcgcaaatgagcctggagaagcgatttggacagtctgctgtttttgttgcttctaccctaatggaaaatggtggtgttcctccttcagcaactccagaaaaccttctcaaagaggctatccatgtcattagttgtggttatgaggataagtcagattggggaatggaggtataatctcatttgaactcctacatgaatctgcattgttctgacatatccactttggcattcactttgtttatattttccgctgtctttcttcagattggatggatctatggttctgtgacagaagatattctgactgggttcaaaatgcatgcccgtggatggcgatccatttactgcatgcctaagcttccagctttcaagggttctgctcctatcaatttttcagatcgtctgaaccaagtgctgaggtgggctttaggttcagttgagattctcttcagtcggcattgtcctatatggtatggttacaatgggaggctaaaatttcttgagaggtttgcgtatgtgaacaccaccatctaccctatcacctccattcctcttctcatgtattgtacattgccagccgtttgtctcttcaccaaccagtttattattcctcaggtttgacacctctctctgtctatctatctctatctctatctctatctctagaacaaaccttaattacgttctgtttaactgaaaccatgttgtgtttgtcatctatttacggttccaaatcctgatcagctggttctattgttcctcttttgcagattagtaacattgcaagtatatggtttctgtctctctttctctccattttcgccacgggtatactagaaatgaggtggagtggcgtaggcatagacgaatggtggagaaacgagcagttttgggtcattggtggagtatccgctcatttattcgctgtgtttcaaggtatcctcaaagtccttgccggtattgacacaaacttcacagttacctcaaaagcttcagatgaagacggagactttgctgagctctacttgttcaaatggacaacacttctgattccgccaacgacgctgctcattgtaaacttagtgggagttgttgcaggagtctcttatgctatcaacagtggataccaatcatggggaccactctttggtaagttgttctttgccttctgggtgattgttcacttgtaccctttcctcaagggtttgatgggtcgacagaaccggactcctaccattgttgtggtctggtctgttctcttggcttctatcttctcgttgttgtgggttaggattgatcccttcactagccgagtcactggcccggacattctggaatgtggaatcaactgttga

SEQ ID NO: 31 - protein, 1065 aa, Arabidopsis thaliana
MESEGETAGKPMKNIVPQTCQICSDNVGKTVDGDRFVACDICSFPVCRPCYEYERKDGNQSCPQCKTRYKRLKGSPAIPGDKDEDGLADEGTVEFNYPQKEKISERMLGWHLTRGKGEEMGEPQYDKEVSHNHLPRLTSRQDTSGEFSAASPERLSVSSTIAGGKRLPYSSDVNQSPNRRIVDPVGLGNVAWKERVDGWKMKQEKNTGPVSTQAASERGGVDIDASTDILADEALLNDEARQPLSRKVSIPSSRINPYRMVIMLRLVILCLFLHYRITNPVPNAFALWLVSVICEIWFALSWILDQFPKWFPVNRETYLDRLALRYDREGEPSQLAAVDIFVSTVDPLKEPPLVTANTVLSILAVDYPVDKVSCYVSDDGAAMLSFESLAETSEFARKWVPFCKKYSIEPRAPEWYFAAKIDYLKDKVQTSFVKDRRAMKREYEEFKIRINALVSKALKCPEEGWVMQDGTPWPGNNTRDHPGMIQVFLGQNGGLDAEGNELPRLVYVSREKRPGFQHHKKAGAMNALVRVSAVLTNGPFILNLDCDHYINNSKALREAMCFLMDPNLGKQVCYVQFPQRFDGIDKNDRYANRNTVFFDINLRGLDGIQGPVYVGTGCVFNRTALYGYEPPIKVKHKKPSLLSKLCGGSRKKNSKAKKESDKKKSGRHTDSTVPVFNLDDIEEGVEGAGFDDEKALLMSQMSLEKRFGQSAVFVASTLMENGGVPPSATPENLLKEAIHVISCGYEDKSDWGMEIGWIYGSVTEDILTGFKMHARGWRSIYCMPKLPAFKGSAPINFSDRLNQVLRWALGSVEILFSRHCPIWYGYNGRLKFLERFAYVNTTIYPITSIPLLMYCTLPAVCLFTNQFIIPQISNIASIWFLSLFLSIFATGILEMRWSGVGIDEWWRNEQFWVIGGVSAHLFAVFQGILKVLAGIDTNFTVTSKASDEDGDFAELYLFKWTTLLIPPTTLLIVNLVGVVAGVSYAINSGYQSWGPLFGKLFFAFWVIVHLYPFLKGLMGRQNRTPTIVVVWSVLLASIFSLLWVRIDPFTSRVTGPDILECGINC

SEQ ID NO: 32 - DNA, 4690 bp, Arabidopsis thaliana
atggaatccgaaggagaaaccgcggtatgcttttttgactcttgcttcatcattatacttacctttatcgaaatcaggaattatatgtactgaaattgattgatttgggtgttgaattgtgtattggagagatctgatttcaaattttctgttgaggtttctaattttggcttcattgattcgacttgatttgtagggaaagccgatgaagaacattgttccgcagacttgccagatctgtagtgacaatgttggcaagactgttgatggagatcgttttgtggcttgtgatatttgttcattcccagtttgtcggccttgctacgagtatgagaggaaagatgggaatcaatcttgtcctcagtgcaaaaccagatacaagaggctcaaaggttctcttttgatccttctgaagtatactgtcttcattgttcatcgatagtttatcagtatgttttgaattttggatcagattggtatttatagcaatttgctaatttctgattctaggtagtcctgctattcctggtgataaagacgaggatggcttagctgatgaaggtactgttgagttcaactaccctcagaaggagaaaatttcagagcggatgcttggttggcatcttactcgtgggaagggagaggaaatgggggaaccccagtatgataaagaggtctctcacaatcatcttcctcgtctcacgagcagacaagatgtaaggcattgctgttcattcttccctcttaagcattcgcatcctcacgcaatttagttttggaatctgattttgtcatttgcttatttacagacttcaggagagttttctgctgcctcacctgaacgcctctctgtatcttctactatcgctgggggaaagcgccttccctattcatcagatgtcaatcaatcacgtaaatatcctttatttctaactctctcgccaacacatatatttgtacctaggcttctcttttatgtcaaaactctaaacaataaaatctgttgttgtcattcacgctgcagcaaatagaaggattgtggatcctgttggactcgggaatgtagcttggaaggagagagttgatggctggaaaatgaagcaagagaagaatactggtcctgtcagcacgcaggctgcttctgaaagaggtggagtagatattgatgccagcacagatatcctagcagatgaggctctgctgtgagttcttgttttgtaatcttgtttgttctgtcgtggtgtaccgagcgtttttcctattaagcaatgtcctgatactcattttccaattctttatttattgtacaggaatgacgaagcgaggcagcctctgtcaaggaaagtttcaattccttcatcacggatcaatccttacagaatggttattatgctgcggcttgttatcctttgtctcttcttgcattaccgtataacaaacccagtgccaaatgcctttgctctatggctggtctctgtgatatgtgagatctggtttgccttatcctggattttggatcagtttcccaagtggtttcctgtgaaccgtgaaacctacctcgacaggcttgctttaaggtaagttctatttccccattcttctgaagcaattactcaaaggattgtttgcctatactgtttcccattttaatttgatcatggtcaatttttgggacagatatgatcgtgaaggtgagccatcacagttagctgctgttgacattttcgtgagtactgttgaccccttgaaggagccaccccttgtgacagccaacacagtgctctctattctggctgttgactacccagttgacaaggtgtcctgttatgtttttgatgatggtgctgctatgttatcatttgaatcacttgcagaaacatcagagtttgctcgtaaatgggtaccattttgcaagaaatatagcatagagcctcgtgcaccagaatggtactttgctgcgaaaatagattacttgaaggataaagttcagacatcatttgtcaaagatcgtagagctatgaaggtaagtttgtagttttagtcatctagtcaccctcactttgattttagtgtatgctatattgaccttttattttctttcagagggaatatgaggaatttaaaatccgaatcaatgcacttgtttccaaagccctaaaatgtcctgaagaagggtgggttatgcaagatggcacaccgtggcctggaaataatacaagggaccatccaggaatgatccaggtaagaaattggttttaactatggaatcgagaatgctctctctttctctctagaagttcattattgaagtaccatttgctgaatgcaggtcttcttagggcaaaatggtggacttgatgcagagggcaatgagctcccgcgtttggtatatgtttctcgagaaaagcgaccaggattccagcaccacaaaaaggctggtgctatgaatgcactggtaagtttctgatcttggatttttgacttcttcattctgaccaatttgttagtctaatctgggtacttttcaaatgaataggtgagagtttcagcagttcttaccaatggacctttcatcttgaatcttgattgtgatcattacataaataacagcaaagccttaagagaagcaatgtgcttcctgatggacccaaacctcgggaagcaagtttgttatgttcagttcccacaaagatttgatggtatcgataagaacgatagatatgctaatcgtaataccgtgttctttgatgtaagtcacacttacctatacttgcgtctaattttcttgttctttcaaattgcttttagacacgaatatacattaaactcacagtttcttgagtttgtcgtaatttttccatgatatgttttccagattaacttgagaggtttagatgggattcaaggacctgtatatgtcggaactggatgtgttttcaacagaacagcattatacggttatgaacctccaataaaagtaaaacacaagaagccaagtcttttatctaagctctgtggtggatcaagaaagaagaattccaaagctaagaaagagtcggacaaaaagaaatcaggcaggcatactgactcaactgttcctgtattcaacctcgatgacatagaagagggagttgaaggtacaactgtttttatttcttctttggtttccgttatacccatatgttgctgtttgaaatattgatccaggggaggggattatttatagttgacagttgtctaaatagtttccatactaggtatctcatcatgtcttaactatttggcatttgtgaaacttaggtgctggttttgatgatgaaaaggcgctcttaatgtcgcaaatgagcctggagaagcgatttggacagtctgctgtttttgttgcttctaccctaatggaaaatggtggtgttcctccttcagcaactccagaaaaccttctcaaagaggctatccatgtcattagttgtggttatgaggataagtcagattggggaatggaggtataatctcatttgaactcctacatgaatctgcattgttctgacatatccactttggcattcactttgtttatattttccgctgtctttcttcagattggatggatctatggttctgtgacagaagatattctgactgggttcaaaatgcatgcccgtggatggcgatccatttactgcatgcctaagcttccagctttcaagggttctgctcctatcaatctttcagatcgtctgaaccaagtgctgaggtgggctttaggttcagttgagattctcttcagtcggcattgtcctatatggtatggttacaatgggaggctaaaatttcttgagaggtttgcgtatgtgaacaccaccatctaccctatcacctccattcctcttctcatgtattgtacattgccagccgtttgtctcttcaccaaccagtttattattcctcaggtttgacacctctctctgtctatctatctctatctctatctctatctctagaacaaaccttaattacgttctgtttaactgaaaccatgttgtgtttgtcatctatttacggttccaaatcctgatcagctggttctattgttcctcttttgcagattagtaacattgcaagtatatggtttctgtctctctttctctccattttcgccacgggtatactagaaatgaggtggagtggcgtaggcatagacgaatggtggagaaacgagcagttttgggtcattggtggagtatccgctcatttattcgctgtgtttcaaggtatcctcaaagtccttgccggtattgacacaaacttcacagttacctcaaaagcttcagatgaagacggagactttgctgagctctacttgttcaaatggacaacacttctgattccgccaacgacgctgctcattgtaaacttagtgggagttgttgcaggagtctcttatgctatcaacagtggataccaatcatggggaccactctttggtaagttgttctttgccttctgggtgattgttcacttgtaccctttcctcaagggtttgatgggtcgacagaaccggactcctaccattgttgtggtctggtctgttctcttggcttctatcttctcgttgttgtgggttaggattgatcccttcactagccgagtcactggcccggacattctggaatgtggaatcaactgttga

SEQ ID NO: 33 - protein, 1065 aa, Arabidopsis thaliana
MESEGETAGKPMKNIVPQTCQICSDNVGKTVDGDRFVACDICSFPVCRPCYEYERKDGNQSCPQCKTRYKRLKGSPAIPGDKDEDGLADEGTVEFNYPQKEKISERMLGWHLTRGKGEEMGEPQYDKEVSHNHLPRLTSRQDTSGEFSAASPERLSVSSTIAGGKRLPYSSDVNQSPNRRIVDPVGLGNVAWKERVDGWKMKQEKNTGPVSTQAASERGGVDIDASTDILADEALLNDEARQPLSRKVSIPSSRINPYRMVIMLRLVILCLFLHYRITNPVPNAFALWLVSVICEIWFALSWILDQFPKWFPVNRETYLDRLALRYDREGEPSQLAAVDIFVSTVDPLKEPPLVTANTVLSILAVDYPVDKVSCYVFDDGAAMLSFESLAETSEFARKWVPFCKKYSIEPRAPEWYFAAKIDYLKDKVQTSFVKDRRAMKREYEEFKIRINALVSKALKCPEEGWVMQDGTPWPGNNTRDHPGMIQVFLGQNGGLDAEGNELPRLVYVSREKRPGFQHHKKAGAMNALVRVSAVLTNGPFILNLDCDHYINNSKALREAMCFLMDPNLGKQVCYVQFPQRFDGIDKNDRYANRNTVFFDINLRGLDGIQGPVYVGTGCVFNRTALYGYEPPIKVKHKKPSLLSKLCGGSRKKNSKAKKESDKKKSGRHTDSTVPVFNLDDIEEGVEGAGFDDEKALLMSQMSLEKRFGQSAVFVASTLMENGGVPPSATPENLLKEAIHVISCGYEDKSDWGMEIGWIYGSVTEDILTGFKMHARGWRSIYCMPKLPAFKGSAPINLSDRLNQVLRWALGSVEILFSRHCPIWYGYNGRLKFLERFAYVNTTIYPITSIPLLMYCTLPAVCLFTNQFIIPQISNIASIWFLSLFLSIFATGILEMRWSGVGIDEWWRNEQFWVIGGVSAHLFAVFQGILKVLAGIDTNFTVTSKASDEDGDFAELYLFKWTTLLIPPTTLLIVNLVGVVAGVSYAINSGYQSWGPLFGKLFFAFWVIVHLYPFLKGLMGRQNRTPTIVVVWSVLLASIFSLLWVRIDPFTSRVTGPDILECGINC

SEQ ID NO: 34 - DNA, 4690 bp, Arabidopsis thaliana
atggaatccgaaggagaaaccgcggtatgcttttttgactcttgcttcatcattatacttacctttatcgaaatcaggaattatatgtactgaaattgattgatttgggtgttgaattgtgtattggagagatctgatttcaaattttctgttgaggtttctaattttggcttcattgattcgacttgatttgtagggaaagccgatgaagaacattgttccgcagacttgccagatctgtagtgacaatgttggcaagactgttgatggagatcgttttgtggcttgtgatatttgttcattcccagtttgtcggccttgctacgagtatgagaggaaagatgggaatcaatcttgtcctcagtgcaaaaccagatacaagaggctcaaaggttctcttttgatccttctgaagtatactgtcttcattgttcatcgatagtttatcagtatgttttgaattttggatcagattggtatttatagcaatttgctaatttctgattctaggtagtcctgctattcctggtgataaagacgaggatggcttagctgatgaaggtactgttgagttcaactaccctcagaaggagaaaatttcagagcggatgcttggttggcatcttactcgtgggaagggagaggaaatgggggaaccccagtatgataaagaggtctctcacaatcatcttcctcgtctcacgagcagacaagatgtaaggcattgctgttcattcttccctcttaagcattcgcatcctcacgcaatttagttttggaatctgattttgtcatttgcttatttacagacttcaggagagttttctgctgcctcacctgaacgcctctctgtatcttctactatcgctgggggaaagcgccttccctattcatcagatgtcaatcaatcacgtaaatatcctttatttctaactctctcgccaacacatatatttgtacctaggcttctcttttatgtcaaaactctaaacaataaaatctgttgttgtcattcacgctgcagcaaatagaaggattgtggatcctgttggactcgggaatgtagcttggaaggagagagttgatggctggaaaatgaagcaagagaagaatactggtcctgtcagcacgcaggctgcttctgaaagaggtggagtagatattgatgccagcacagatatcctagcagatgaggctctgctgtgagttcttgttttgtaatcttgtttgttctgtcgtggtgtaccgagcgtttttcctattaagcaatgtcctgatactcattttccaattctttatttattgtacaggaatgacgaagcgaggcagcctctgtcaaggaaagtttcaattccttcatcacggatcaatccttacagaatggttattatgctgcggcttgttatcctttgtctcttcttgcattaccatataacaaacccagtgccaaatgcctttgctctatggctggtctctgtgatatgtgagatctggtttgccttatcctggattttggatcagtttcccaagtggtttcctgtgaaccgtgaaacctacctcgacaggcttgctttaaggtaagttctatttccccattcttctgaagcaattactcaaaggattgtttgcctatactgtttcccattttaatttgatcatggtcaatttttgggacagatatgatcgtgaaggtgagccatcacagttagctgctgttgacattttcgtgagtactgttgaccccttgaaggagccaccccttgtgacagccaacacagtgctctctattctggctgttgactacccagttgacaaggtgtcctgttatgtttctgatgatggtgctgctatgttatcatttgaatcacttgcagaaacatcagagtttgctcgtaaatgggtaccattttgcaagaaatatagcatagagcctcgtgcaccagaatggtactttgctgcgaaaatagattacttgaaggataaagttcagacatcatttgtcaaagatcgtagagctatgaaggtaagtttgtagttttagtcatctagtcaccctcactttgattttagtgtatgctatattgaccttttattttctttcagagggaatatgaggaatttaaaatccgaatcaatgcacttgtttccaaagccctaaaatgtcctgaagaagggtgggttatgcaagatggcacaccgtggcctggaaataatacaagggaccatccaggaatgatccaggtaagaaattggttttaactatggaatcgagaatgctctctctttctctctagaagttcattattgaagtaccatttgctgaatgcaggtcttcttagggcaaaatggtggacttgatgcagagggcaatgagctcccgcgtttggtatatgtttctcgagaaaagcgaccaggattccagcaccacaaaaaggctggtgctatgaatgcactggtaagtttctgatcttggatttttgacttcttcattctgaccaatttgttagtctaatctgggtacttttcaaatgaataggtgagagtttcagcagttcttaccaatggacctttcatcttgaatcttgattgtgatcattacataaataacagcaaagccttaagagaagcaatgtgcttcctgatggacccaaacctcgggaagcaagtttgttatgttcagttcccacaaagatttgatggtatcgataagaacgatagatatgctaatcgtaataccgtgttctttgatgtaagtcacacttacctatacttgcgtctaattttcttgttctttcaaattgcttttagacacgaatatacattaaactcacagtttcttgagtttgtcgtaatttttccatgatatgttttccagattaacttgagaggtttagatgggattcaaggacctgtatatgtcggaactggatgtgttttcaacagaacagcattatacggttatgaacctccaataaaagtaaaacacaagaagccaagtcttttatctaagctctgtggtggatcaagaaagaagaattccaaagctaagaaagagtcggacaaaaagaaatcaggcaggcatactgactcaactgttcctgtattcaacctcgatgacatagaagagggagttgaaggtacaactgtttttatttcttctttggtttccgttatacccatatgttgctgtttgaaatattgatccaggggaggggattatttatagttgacagttgtctaaatagtttccatactaggtatctcatcatgtcttaactatttggcatttgtgaaacttaggtgctggttttgatgatgaaaaggcgctcttaatgtcgcaaatgagcctggagaagcgatttggacagtctgctgtttttgttgcttctaccctaatggaaaatggtggtgttcctccttcagcaactccagaaaaccttctcaaagaggctatccatgtcattagttgtggttatgaggataagtcagattggggaatggaggtataatctcatttgaactcctacatgaatctgcattgttctgacatatccactttggcattcactttgtttatattttccgctgtctttcttcagattggatggatctatggttctgtgacagaagatattctgactgggttcaaaatgcatgcccgtggatggcgatccatttactgcatgcctaagcttccagctttcaagggttctgctcctatcaatctttcagatcgtctgaaccaagtgctgaggtgggctttaggttcagttgagattctcttcagtcggcattgtcctatatggtatggttacaatgggaggctaaaatttcttgagaggtttgcgtatgtgaacaccaccatctaccctatcacctccattcctcttctcatgtattgtacattgccagccgtttgtctcttcaccaaccagtttattattcctcaggtttgacacctctctctgtctatctatctctatctctatctctatctctagaacaaaccttaattacgttctgtttaactgaaaccatgttgtgtttgtcatctatttacggttccaaatcctgatcagctggttctattgttcctcttttgcagattagtaacattgcaagtatatggtttctgtctctctttctctccattttcgccacgggtatactagaaatgaggtggagtggcgtaggcatagacgaatggtggagaaacgagcagttttgggtcattggtggagtatccgctcatttattcgctgtgtttcaaggtatcctcaaagtccttgccggtattgacacaaacttcacagttacctcaaaagcttcagatgaagacggagactttgctgagctctacttgttcaaatggacaacacttctgattccgccaacgacgctgctcattgtaaacttagtgggagttgttgcaggagtctcttatgctatcaacagtggataccaatcatggggaccactctttggtaagttgttctttgccttctgggtgattgttcacttgtaccctttcctcaagggtttgatgggtcgacagaaccggactcctaccattgttgtggtctggtctgttctcttggcttctatcttctcgttgttgtgggttaggattgatcccttcactagccgagtcactggcccggacattctggaatgtggaatcaactgttga

SEQ ID NO: 35 - protein, 1065 aa, Arabidopsis thaliana
MESEGETAGKPMKNIVPQTCQICSDNVGKTVDGDRFVACDICSFPVCRPCYEYERKDGNQSCPQCKTRYKRLKGSPAIPGDKDEDGLADEGTVEFNYPQKEKISERMLGWHLTRGKGEEMGEPQYDKEVSHNHLPRLTSRQDTSGEFSAASPERLSVSSTIAGGKRLPYSSDVNQSPNRRIVDPVGLGNVAWKERVDGWKMKQEKNTGPVSTQAASERGGVDIDASTDILADEALLNDEARQPLSRKVSIPSSRINPYRMVIMLRLVILCLFLHYHITNPVPNAFALWLVSVICEIWFALSWILDQFPKWFPVNRETYLDRLALRYDREGEPSQLAAVDIFVSTVDPLKEPPLVTANTVLSILAVDYPVDKVSCYVSDDGAAMLSFESLAETSEFARKWVPFCKKYSIEPRAPEWYFAAKIDYLKDKVQTSFVKDRRAMKREYEEFKIRINALVSKALKCPEEGWVMQDGTPWPGNNTRDHPGMIQVFLGQNGGLDAEGNELPRLVYVSREKRPGFQHHKKAGAMNALVRVSAVLTNGPFILNLDCDHYINNSKALREAMCFLMDPNLGKQVCYVQFPQRFDGIDKNDRYANRNTVFFDINLRGLDGIQGPVYVGTGCVFNRTALYGYEPPIKVKHKKPSLLSKLCGGSRKKNSKAKKESDKKKSGRHTDSTVPVFNLDDIEEGVEGAGFDDEKALLMSQMSLEKRFGQSAVFVASTLMENGGVPPSATPENLLKEAIHVISCGYEDKSDWGMEIGWIYGSVTEDILTGFKMHARGWRSIYCMPKLPAFKGSAPINLSDRLNQVLRWALGSVEILFSRHCPIWYGYNGRLKFLERFAYVNTTIYPITSIPLLMYCTLPAVCLFTNQFIIPQISNIASIWFLSLFLSIFATGILEMRWSGVGIDEWWRNEQFWVIGGVSAHLFAVFQGILKVLAGIDTNFTVTSKASDEDGDFAELYLFKWTTLLIPPTTLLIVNLVGVVAGVSYAINSGYQSWGPLFGKLFFAFWVIVHLYPFLKGLMGRQNRTPTIVVVWSVLLASIFSLLWVRIDPFTSRVTGPDILECGINC

SEQ ID NO: 36 - DNA, 4779 bp, Arabidopsis thaliana
atgaacaccggtggtcggttaatcgccggttctcacaacaggaatgagtttgtcctcattaatgccgatgagaatgcccgagtatgtttctcctcttcttttgtttccaattctctgtcttttgatctgtgtttctctatctctgttcaaaagtctctgactttttttacttttcttgtggatctggctcttaccactgcaaatcaattaagatttagggtttttagtactagtattaagattacgtacccttgtagctaattttatcaagaattgattgtgtcggtgggatggatttttccggatttgacttgtcttaattctccaatttaagagatttcttcaattgcaattatgaatctatcaatgtgaagagtaataattatgttattgggttactttgatctggtgtgagatccagtctgatagtgtcactactatgatctgatgtatttaactctactgttttgtgcagataagatcagtccaagagctgagtggacagacatgtcaaatctgcagagatgagatcgaattgactgttgatggagaaccgtttgtggcatgtaacgaatgtgcattccctgtgtgtagaccttgctatgagtacgaaagacgagaaggcaatcaagcttgtccacagtgcaaaacccgtttcaaacgtcttaaaggttcgttgtttgttagaccaaatttctttggttttttgtgaatgtagaagattttctgatttgttcggcctatgttgttgtttgttaggaagtccaagagttgaaggtgatgaagaggaagatgacattgatgatttagacaatgagtttgagtatggaaataatgggattggatttgatcaggtttctgaaggtatgtcaatctctcgtcgcaactccggtttcccacaatctgatttggattcagctccacctggctctcagattccattgctgacttacggcgacgaggtaaaaatctcagaatgtatccacattgtataacccatcttcagtaattggctcactcagatttctcttttgttttattacaggacgttgagatttcttctgatagacatgctcttattgttcctccttcacttggtggtcatggcaatagagttcatcctgtttctctttctgacccgaccgtggctgcacatccaaggcctatggtacctcagaaagatcttgcggtttatggttatggaagtgtcgcttggaaagatcggatggaggaatggaagagaaagcagaatgagaaacttcaggttgttaggcatgaaggagatcctgattttgaagatggtgatgatgctgattttccaatgtaaggcaaagaatataattttttttgttgatgtcttgttccgttgcagtgatatttatcaagccttttttttccattttaggatggatgagggaaggcagccattgtctaggaagataccaatcaaatcgagcaagataaatccttaccggatgttaattgtgctacgtcttgtgattcttggtctcttctttcactaccgtattcttcaccccgtcaaagatgcatatgctttgtggcttatttctgttatatgtgagatatggtttgctgtttcatgggttcttgatcagttccctaaatggtaccctatcgagcgagaaacgtacttggaccgactctcattaaggtacttacatcttgtgggttattacacttggaaatgttaaaactttgttttggggatataatccttattttttttgtttgcagatatgagaaagaagggaaaccgtcgggactatcccctgtggatgtatttgttagtacagtggatccattgaaagagcctccgcttattactgcaaatactgtcttgtctattcttgctgttgattatcctgtcgataaggttgcttgttacgtatctgatgatggtgctgctatgcttactttcgaagctctttctgagaccgctgaattcgcaaggaaatgggttcctttctgcaagaaatattgtattgagcctcgtgctcccgaatggtatttctgccataaaatggactacttgaagaataaagttcatcccgcatttgttagggagcggcgagccatgaaggttactagttcttacttttttataaatttgatttgatgagaaaagttttggtctaattgattcttgctttagaaaaaaaaaattcatgagaaaagttatcaatcttttgttatatgggctcttatgaaagaagatggtggctttgaaaattgatttgaaagattgtgtgttttactggttttgacagagagattatgaagaattcaaagtaaagatcaatgctttagtagcaacagcacagaaagtgcctgaggatggttggactatgcaagacggtacaccttggcccggtaatagtgtgcgagatcatcctggcatgattcaggtgagtttcaaatgcttcttatttctgaaaagccttcttatgtgttgtccttcaaaatttaattatactttgttttcttgttaaaggtcttccttggaagtgacggtgttcgtgatgtcgaaaacaacgagttgcctcgattagtttacgtttctcgtgagaagagacccggatttgatcaccataagaaggctggagctatgaattccctggtaaatgatatactttttaaagctctaaaccttcttctttgtaaattacgtcttgccatttattgaaatggttcctgactcttgatttcatctacaaaacttttgttgaagatacgagtctctggggttctatcaaatgctccttaccttctgaatgtcgattgtgatcactacatcaacaatagcaaagctcttagagaagcaatgtgtttcatgatggatcctcagtcaggaaagaaaatctgttatgttcagttccctcaaaggttcgatgggattgataggcacgatcgatactcaaatcgcaatgttgtgttctttgatgtaagtacagccaccactttcctattgtatccctttttcttgagatttctgtagaataccaactaatgaatctttatttacagatcaatatgaaaggtttggatgggctacaagggcctatatacgtcggtacaggttgtgttttcaggaggcaagcgctttacggatttgatgcaccgaagaagaagaagggcccacgtaagacatgcaattgctggccaaaatggtgtctcctatgttttggttcaagaaagaatcgtaaagcaaagacagtggctgcggataagaagaagaagaatagggaagcgtcaaagcagatccacgcattagaaaatatcgaagagggccgcgtcactaaaggtatcatacaaatcctgtttgttgttaaactctttcgttagtcggtgcattttactaaaaaaataaaatttaaaaaacattctaggttctaacgtagaacagtcaaccgaggcaatgcaaatgaagttggagaagaaatttgggcagtctcctgtatttgttgcatctgcgcgtatggagaatggtgggatggctagaaacgcaagcccggcttgtctgcttaaagaagccatccaagtcattagttgcggatatgaagataaaactgaatggggaaaagaggtaagcagccggttttaaacctttgttgtgtttattcaatcaattcttgattttgatgatgaccttgtgaaaaaaatctcagattgggtggatctatggttctgttaccgaagatattcttacgggttttaagatgcattctcatggttggagatctgtttattgtacaccaaagttagcggctttcaaaggatcagctccaatcaatctttcggatcgtctccatcaagttcttcgatgggcgcttgggtcggttgagattttcttgagtaggcattgtcctatttggtatggttatggaggtgggttgaaatggcttgagcggttgtcctacattaactctgtggtttacccgtggacctctctaccgctcatcgtttactgttctctccctgccatctgtcttctcactggaaaattcatcgttcccgaggtaaaacaatcatcttgagttctcaaaatatgaatctttatttcacgttttgtgcttattcattttccttgccactgggggttaaaagtatcatatgaatctttattccaagttgtgtgttttaagaccggaaaacgattcttgttccttctttttccagattagcaactatgcgagtatcctcttcatggcgctcttctcgtcgattgcaataacgggtattctcgagatgcaatggggcaaagttgggatcgatgattggtggagaaacgaacagttttgggtcattggaggtgtttctgcgcatctgtttgctctcttccaaggtctcctcaaggttcttgctggtgtcgacactaacttcacagtcacatcaaaagcagctgatgatggagagttctctgacctttacctcttcaaatggacttcacttctcatccctccaatgactctactcatcataaacgtcattggagtcatagtcggagtctttgatgccatcagcaatggatacgactcgtggggaccgcttttcggaagactgttctttgcactttgggtcatcattcatctttacccgttccttaaaggtttgcttgggaaacaagatagaatgccaaccattattgtcgtctggtccatcctcctggcctcgattcttacacttctttgggtccgggttaatccgtttgtggcgaaaggcggtcctattctcgagatctgtggtttagactgcttgtga

SEQ ID NO: 37 - protein, 1084 aa, Arabidopsis thaliana
MNTGGRLIAGSHNRNEFVLINADENARIRSVQELSGQTCQICRDEIELTVDGEPFVACNECAFPVCRPCYEYERREGNQACPQCKTRFKRLKGSPRVEGDEEEDDIDDLDNEFEYGNNGIGFDQVSEGMSISRRNSGFPQSDLDSAPPGSQIPLLTYGDEDVEISSDRHALIVPPSLGGHGNRVHPVSLSDPTVAAHPRPMVPQKDLAVYGYGSVAWKDRMEEWKRKQNEKLQVVRHEGDPDFEDGDDADFPMMDEGRQPLSRKIPIKSSKINPYRMLIVLRLVILGLFFHYRILHPVKDAYALWLISVICEIWFAVSWVLDQFPKWYPIERETYLDRLSLRYEKEGKPSGLSPVDVFVSTVDPLKEPPLITANTVLSILAVDYPVDKVACYVSDDGAAMLTFEALSETAEFARKWVPFCKKYCIEPRAPEWYFCHKMDYLKNKVHPAFVRERRAMKRDYEEFKVKINALVATAQKVPEDGWTMQDGTPWPGNSVRDHPGMIQVFLGSDGVRDVENNELPRLVYVSREKRPGFDHHKKAGAMNSLIRVSGVLSNAPYLLNVDCDHYINNSKALREAMCFMMDPQSGKKICYVQFPQRFDGIDRHDRYSNRNVVFFDINMKGLDGLQGPIYVGTGCVFRRQALYGFDAPKKKKGPRKTCNCWPKWCLLCFGSRKNRKAKTVAADKKKKNREASKQIHALENIEEGRVTKGSNVEQSTEAMQMKLEKKFGQSPVFVASARMENGGMARNASPACLLKEAIQVISCGYEDKTEWGKEIGWIYGSVTEDILTGFKMHSHGWRSVYCTPKLAAFKGSAPINLSDRLHQVLRWALGSVEIFLSRHCPIWYGYGGGLKWLERLSYINSVVYPWTSLPLIVYCSLPAICLLTGKFIVPEISNYASILFMALFSSIAITGILEMQWGKVGIDDWWRNEQFWVIGGVSAHLFALFQGLLKVLAGVDTNFTVTSKAADDGEFSDLYLFKWTSLLIPPMTLLIINVIGVIVGVFDAISNGYDSWGPLFGRLFFALWVIIHLYPFLKGLLGKQDRMPTIIVVWSILLASILTLLWVRVNPFVAKGGPILEICGLDCL